European Patent Application EP 4 317 416 A1, published February 7, 2024. Title: Recombinant microorganism and production method of C6 compounds. Applicant: Asahi Kasei Corporation. The sequence listing filed with the application follows.

SEQUENCE LISTING (251 sequences)

SEQ ID NO: 1 - protein, 401 aa, Escherichia coli
MREAFICDGIRTPIGRYGGALSSVRADDLAAIPLRELLVRNPRLDAECIDDVILGCANQAGEDNRNVARMATLLAGLPQSVSGTTINRLCGSGLDALGFAARAIKAGDGDLLIAGGVESMSRAPFVMGKAASAFSRQAEMFDTTIGWRFVNPLMAQQFGTDSMPETAENVAELLKISREDQDSFALRSQQRTAKAQSSGILAEEIVPVVLKNKKGVVTEIQHDEHLRPETTLEQLRGLKAPFRANGVITAGNASGVNDGAAALIIASEQMAAAQGLTPRARIVAMATAGVEPRLMGLGPVPATRRVLERAGLSIHDMDVIELNEAFAAQALGVLRELGLPDDAPHVNPNGGAIALGHPLGMSGARLALAASHELHRRNGRYALCTMCIGVGQGIAMILERV

SEQ ID NO: 2 - protein, 475 aa, Escherichia coli
MMINVQTVAVIGSGTMGAGIAEVAASHGHQVLLYDISAEALTRAIDGIHARLNSRVTRGKLTAETCERTLKRLIPVTDIHALAAADLVIEAASERLEVKKALFAQLAEVCPPQTLLTTNTSSISITAIAAEIKNPERVAGLHFFNPAPVMKLVEVVSGLATAAEVVEQLCELTLSWGKQPVRCHSTPGFIVNRVARPYYSEAWRALEEQVAAPEVIDAALRDGAGFPMGPLELTDLIGQDVNFAVTCSVFNAFWQERRFLPSLVQQELVIGGRLGKKSGLGVYDWRAEREAVVGLEAVSDSFSPMKVEKKSDGVTEIDDVLLIETQGETAQALAIRLARPVVVIDKMAGKVVTIAAAAVNPDSATRKAIYYLQQQGKTVLQIADYPGMLIWRTVAMIINEALDALQKGVASEQDIDTAMRLGVNYPYGPLAWGAQLGWQRILRLLENLQHHYGEERYRPCSLLRQRALLESGYES

SEQ ID NO: 3 - protein, 255 aa, Escherichia coli
MSELIVSRQQRVLLLTLNRPAARNALNNALLMQLVNELEAAATDTSISVCVITGNARFFAAGADLNEMAEKDLAATLNDTRPQLWARLQAFNKPLIAAVNGYALGAGCELALLCDVVVAGENARFGLPEITLGIMPGAGGTQRLIRSVGKSLASKMVLSGESITAQQAQQAGLVSDVFPSDLTLEYALQLASKMARHSPLALQAAKQALRQSQEVALQAGLAQERQLFTLLAATEDRHEGISAFLQKRTPDFKGR

SEQ ID NO: 4 - DNA, 22 bp, Artificial Sequence
  primer
atgcaaaccatcgaaaacgaag

SEQ ID NO: 5 - protein, 384 aa, Acinetobacter baylyi
MIRDEGMLQQLLSTIRDFVKNELIPREHEVAEKDCIPEDIIQQMRELGLFGLTIPEEYGGLGITMEEEVNVAFELGQTSPAFRSLIGTNNGIGSSGLIIDGTEEQKQKYLPRYASGEIIGSFCLTEPEAGSDAASLKTTAVKDGDFYILNGTKRFITNAPHAATFTVMARTNPAIKGAGGISAFLVEANTPGITLGKIDQKMGQKGSHTCDVIFENCRVPASALIGGVEGVGFKTAMKVLDKGRLHIGAYSVGVAERMLNDALHYAVERKQFGQPIANFQLIQAMLADSKAEIYAAKCMVLDAARRRDEGQNISTEASCAKMFATEMCGRVADRCVQIHGGAGYISEYSIERFYRDVRLFRLYEGTTQVQQIIIAKNMIKEVTS

SEQ ID NO: 6 - protein, 386 aa, Candida tropicalis
MYSVLKQSIRPRLLATHNQFRTMITAQAVLYTQHGEPKDVLFTQSFEIDDDNLAPNEVIVKTLGSPVNPSDINQIQGVYPSKPAKTTGFGTTEPAAPCGNEGLFEVIKVGSNVSSLEAGDWVIPSHVNFGTWRTHALGNDDDFIKLPNPAQSKANGKPNGLTINQGATISVNPLTAYLMLTHYVKLTPGKDWFIQNGGTSAVGKYASQIGKLLNFNSISVIRDRPNLDEVVASLKELGATQVITEDQNNSREFGPTIKEWIKQSGGEAKLALNCVGGKSSTGIARKLNNNGLMLTYGGMSFQPVTIPTSLYIFKNFTSAGFWVTELLKNNKELKTSTLNQIIAWYEEGKLTDAKSIETLYDGTKPLHELYQDGVANSKDGKQLITY

SEQ ID NO: 7 - protein, 364 aa, Candida tropicalis
MITAQAVLYTQHGEPKDVLFTQSFEIDDDNLAPNEVIVKTLGSPVNPSDINQIQGVYPSKPAKTTGFGTTEPAAPCGNEGLFEVIKVGSNVSSLEAGDWVIPSHVNFGTWRTHALGNDDDFIKLPNPAQSKANGKPNGLTINQGATISVNPLTAYLMLTHYVKLTPGKDWFIQNGGTSAVGKYASQIGKLLNFNSISVIRDRPNLDEVVASLKELGATQVITEDQNNSREFGPTIKEWIKQSGGEAKLALNCVGGKSSTGIARKLNNNGLMLTYGGMSFQPVTIPTSLYIFKNFTSAGFWVTELLKNNKELKTSTLNQIIAWYEEGKLTDAKSIETLYDGTKPLHELYQDGVANSKDGKQLITY

SEQ ID NO: 8 - protein, 388 aa, Candida auris
MFVPTVAGKRFLTNQLRKSPQFTRMLTSHAVIFSSHGEPKDVLKTHTYEIDENNIKPNEIVLKTLGAPVNPSDINQVQGVYPSQPEKTTQLGTSEPSAVGGNEGLFEIIKIGSDVKGFQVGDWAIPTSVNFGTWRSHALCEEGKMMKVPNPEQSKQAGKKQGLTINQGATLSVNPLTAYLMLTHYVKLTPGKDWFIQNGGNSAVGKFASQIGKLLGIHSISVVRDRPEIEELKKELKEVCGATQVITEEQNNSKDFGPQVKQWVKETGGEIKLALNCVGGKSSAGVARKLAPNGLMLTYGGMSFQPVTLPTSLHIFKNVTSAGFWVTELLKSDPNLKRETVDKIVEWYTSGELLDAPSKENQWGDQDLAQVFIDAVANSKSGKQLVKF

SEQ ID NO: 9 - protein, 380 aa, Kluyveromyces marxianus
MSSFLSKRFISTTQRAMSQLPKAKSLIYSSHDQDVSKILKVHTYQPKGSAESSILLKTLAFPINPSDINQLEGVYPSKPEKVLDYSTEEPSAIAGNEGLFEVVSVPSGVKNLKAGDRVIPLQANFGTWSTYRTCESENDLIKIEGVDLYTAATIAVNGCTAYQMVNDYIEWDPSGNDWLVQNAGTSSVSKIVTQIAKDKGIKTLSVVRDRDNFDEVAEKLEKKYGATKVISESQNGEREFGNEVLPKILGPNAQVKLALNSVGGKSCTNIARKLSPNGLMLTYGGMSKQPVTLPTGLFIFNSIRSHGFWVTANSKRDPENKRKTVDAVVKLYRDGKIISPKEDIRTLEWDVNNLSDEGVLDLVNRGIATKGAKNMVVLKW

SEQ ID NO: 10 - protein, 373 aa, Pichia kudriavzevii
MSLRSVFSVSSIRRMSSITARAIVYNAHGEPKDTLKCHSYKIDLQNLQPNEVVVQTLAAPLNPSDINQIQGVYPSKPPLSIDSLPELKEPAAVTGNEGVFKVIAKGSNVGELETGDWCIPSGVNFGTWCTHRLTTDKNLLKMPKTISLNQAATIAVNPSSAYQMLTHFVKLQPGDWFIQNGANSQVGRAAIQIGHKLGYKSLNIVRNRDNLDELVKDLESIGATKVITEDESASKEFGATVKEWLEGKEIKLGLNCIGGPSASNLARKLGHDATILTYGAMSKKPLSLPTGNFIFKNLTAKGFWITGNIKRHPELRIETINAVLKFMEDGTLKEPKVNEPKVKLSTTTNESFLETVLAALEDSQKGKQLLKFE

SEQ ID NO: 11 - protein, 448 aa, Thermothelomyces thermophilus
MASVLSPNAAARHLLRPATRSTPPRLLPSAILHQSGNNSTRNPRISDPQSIAQRLGRRYKSGPYGYTQAKTLVFSRFGEPSDVLRLHTHSISPTLPDGAVLVRALAAPVNPADVNTIQGTYGARPAFSPLLGTPEPSAVPGNEGCFEVVAVGPRVGGGLRKGDWVIPATTGFGTFRTHALVENADRALLRVGGDKGTAGLTAKQVATVSVNPCSAYRMLKDYVDLVDLSVKSFARGDGATGGAWFLQNGANSGVGRAAIQLGRLWGLRSINVVRERATAEETEALKSELRELGATVVVTEAEFLDRSFSARLKEEWTRGDREPVMLGLNCVGGKSASAMIKALSPKGCMVTYGGMSRQSFPFPTGPQIFKRLRFEGFWLSEWAKENPAEKRNTINEILELMREGKFKESPFKEVEWNWDTEEKVLKDAIQGTLEGFKSGKGLFVFGDT

SEQ ID NO: 12 - protein, 443 aa, Thermothielavioides terrestris
MASALNPRHLPLRLALRPRLPLLPSTSSTTTTTTPPSCLPIPTSIRLPPRRHKSGPYGYTLAKTLVFSRFGEPRDVLSLHTHSISPALPDGAALLRALAAPVNPADVNTVQGTYGAKPAFERLLGTPEPAAVPGNEGCFEVVAIGGGAGGGGGLKKGDWVIPAQSGFGTFRTHALVEGAERKLIRVGGAKGREGLRAAQVATVSVNPCSAYRMLRDYVDLVDLSVQSFARGDGATGGAWFVQNGANSGVGRAAIQLGRLWGLRSINVVRERATPEETAALKRELAELGATVVVTESEFLDRSFADRLRDEWTRGGREPVMLGLNCVGGKSAAAMVKALSPRGCMVTYGGMSRQSFPFPTGQQIFKRLRFEGFWLSEWAKENPAAKRDTINEILELMREGKFKEAPLQEVEWNWDTEESVLKDTIQGTLEGFRPGKSIFVFKDT

SEQ ID NO: 13 - protein, 439 aa, Chaetomium thermophilum
MASILSPHSALRLGGISTLSRQTLLRTSRVTLTQLPKTAPQLPQRRHKSAPYGYTQSKTLVFPRFGEPIDVLSLHTHSISPTLPDTAVLLRTLAAPINPADVNTIQGTYGAKPTFSNLLGTAEPAAVPGNEGVFEVVSVGSEIAKRGVFKKGDWVIPSSSGFGTFRTHVLVEEAEQKLWRIGGEKGTEGLTPVQVATVSVNPCSAYRMLRDYVDLVGVSVRMYQEGGSDVRGGAWFLQNGANSGVGRAAIQLGRLWGLRSINVVRERATAEETEALKKELYDLGATVVVTESEFLDRSFTQRLNEEWTRGGKEPLLLALNCVGGKSAQQIVRALSPKGTMVTYGGMSRQSFPFPTGPQIFKRLRFEGFWLSEWAKENPAEKKKCVDEIIELMREGKFKEAPVQEIRWDWETEEKVLKEAVQGTLEGFRSGKGVFIFGDT

SEQ ID NO: 14 - protein, 422 aa, Podospora anserina
MAAPRLTSKALRLPTSKLLRPALTTATPRAAPTLTQKRHLTGPYGYHQSKALTFSSFGEPIDVLSLHTHSISPTLPSGSVLVRTLAAPVNPADVNTIQGTYGSKPPFTTLLGTAQPSAVPGNEACFEVLSVGQGVKGLEKGDWVIPAKTGFGTFRTHALVEEAEGKLMRVEREGLTPVQVATVSVNPCSAYRMLKDYVDLVGLSMRWYREGKDVSGGAWFLQNGANSGVGRAAVQFGRLWGLRSINVVRERETPEETEKLKEELTGLGANVVLTEQEFLDRSFRDRLGELTKRGKEPLLLGMNCVGGKSASAVVKALSPKGCMVTYGGMSRQSFPFPTGPQIFKRLRFEGFWLSEWGKENPEGKKKMIEDILNLMREGKFKESPVQEVEWNWETEEKTLKEAVQGTLGGFRSGKGVFVFGET

SEQ ID NO: 15 - protein, 424 aa, Purpureocillium lilacinum
MASSRLLGPPLRLPSSGFSRPVAALNCRAAALPLHLPRTAVRYRSGPYGYTQAKALVYSKNGEPADVLKLHTHSISPSIPSTSVLVRCLAAPINPADVNTIQGTYGSKQPLTSLIGTSEPSAVPGNEGVFEVLSAGSPSSELKKGDWVIPAASQIGTWRTHAVFGADELLKVDKEGLTPTQVSLVSVNPCTAYRILRSYGPSAGVKAALGMRPLEVGSGQWFIQNGANSGVGRAAIQFGKLWGLRSINVIRDRDTVEATDALKQELRDLGADVVVAESEFLSRGWKDQLAEITRKGREQVGLGLNCVGGKSATALARSLGEGATLVSYGGMAKQPVALPVGLLIFKDIRFVGFWLSKWNQQDVVGRRHMVADILGLMRDGKFRDAPVDEVKWDWDTDEATLRGAAQRGLEGFRQGKGVYVFGDT

SEQ ID NO: 16 - protein, 405 aa, Pyrenophora teres
MASKLISPSPRLAQSCLRRTRNLAPVTARFPQRRYISAYGYEQAKALTFTEYGDPSAVLSLHSHSISPPHSNYMTLRFLASPINPADINQIQGVYPSKPTFTTSLGTPNPIAVAGNEGVAEIIALGEGVKKEGFKKGDWVFMKGPGFGTWRTHASATTNDVVKLNDQMREGITAIQAGTVSINPCTAYRMLRDFTTLSEGDWFIQNGANSGVGRAAIQLGRKWGYKSINIIRSREDKNKEEAMKKELHNLGADVVITDAELQAQGIKDQAKEWTNGGRSPIRLALNCVNGKAATAMAKLLSSSAHFVTYGAMSKQPLTIPASMLIFKDIHFHGFWVSRWAEEHPEEKQKTVADVLDMTRKGEFKDMPVDEIKWEWETKGEELVAKVKDTLEGYRDGKGIFVFGKT

SEQ ID NO: 17 - protein, 453 aa, Clostridium kluyveri
MSNEVSIKELIEKAKVAQKKLEAYSQEQVDVLVKALGKVVYDNAEMFAKEAVEETEMGVYEDKVAKCHLKSGAIWNHIKDKKTVGIIKEEPERALVYVAKPKGVVAATTPITNPVVTPMCNAMAAIKGRNTIIVAPHPKAKKVSAHTVELMNAELKKLGAPENIIQIVEAPSREAAKELMESADVVIATGGAGRVKAAYSSGRPAYGVGPGNSQVIVDKGYDYNKAAQDIITGRKYDNGIICSSEQSVIAPAEDYDKVIAAFVENGAFYVEDEETVEKFRSTLFKDGKINSKIIGKSVQIIADLAGVKVPEGTKVIVLKGKGAGEKDVLCKEKMCPVLVALKYDTFEEAVEIAMANYMYEGAGHTAGIHSDNDENIRYAGTVLPISRLVVNQPATTAGGSFNNGFNPTTTLGCGSWGRNSISENLTYEHLINVSRIGYFNKEAKVPSYEEIWG

SEQ ID NO: 18 - protein, 1174 aa, Nocardia iowensis
MAVDSPDERLQRRIAQLFAEDEQVKAARPLEAVSAAVSAPGMRLAQIAATVMAGYADRPAAGQRAFELNTDDATGRTSLRLLPRFETITYRELWQRVGEVAAAWHHDPENPLRAGDFVALLGFTSIDYATLDLADIHLGAVTVPLQASAAVSQLIAILTETSPRLLASTPEHLDAAVECLLAGTTPERLVVFDYHPEDDDQRAAFESARRRLADAGSSVIVETLDAVRARGRDLPAAPLFVPDTDDDPLALLIYTSGSTGTPKGAMYTNRLAATMWQGNSMLQGNSQRVGINLNYMPMSHIAGRISLFGVLARGGTAYFAAKSDMSTLFEDIGLVRPTEIFFVPRVCDMVFQRYQSELDRRSVAGADLDTLDREVKADLRQNYLGGRFLVAVVGSAPLAAEMKTFMESVLDLPLHDGYGSTEAGASVLLDNQIQRPPVLDYKLVDVPELGYFRTDRPHPRGELLLKAETTIPGYYKRPEVTAEIFDEDGFYKTGDIVAELEHDRLVYVDRRNNVLKLSQGEFVTVAHLEAVFASSPLIRQIFIYGSSERSYLLAVIVPTDDALRGRDTATLKSALAESIQRIAKDANLQPYEIPRDFLIETEPFTIANGLLSGIAKLLRPNLKERYGAQLEQMYTDLATGQADELLALRREAADLPVLETVSRAAKAMLGVASADMRPDAHFTDLGGDSLSALSFSNLLHEIFGVEVPVGVVVSPANELRDLANYIEAERNSGAKRPTFTSVHGGGSEIRAADLTLDKFIDARTLAAADSIPHAPVPAQTVLLTGANGYLGRFLCLEWLERLDKTGGTLICVVRGSDAAAARKRLDSAFDSGDPGLLEHYQQLAARTLEVLAGDIGDPNLGLDDATWQRLAETVDLIVHPAALVNHVLPYTQLFGPNVVGTAEIVRLAITARRKPVTYLSTVGVADQVDPAEYQEDSDVREMSAVRVVRESYANGYGNSKWAGEVLLREAHDLCGLPVAVFRSDMILAHSRYAGQLNVQDVFTRLILSLVATGIAPYSFYRTDADGNRQRAHYDGLPADFTAAAITALGIQATEGFRTYDVLNPYDDGISLDEFVDWLVESGHPIQRITDYSDWFHRFETAIRALPEKQRQASVLPLLDAYRNPCPAVRGAILPAKEFQAAVQTAKIGPEQDIPHLSAPLIDKYVSDLELLQLL

SEQ ID NO: 19 - protein, 1174 aa, Mycobacterium marinum
MSPITREERLERRIQDLYANDPQFAAAKPATAITAAIERPGLPLPQIIETVMTGYADRPALAQRSVEFVTDAGTGHTTLRLLPHFETISYGELWDRISALADVLSTEQTVKPGDRVCLLGFNSVDYATIDMTLARLGAVAVPLQTSAAITQLQPIVAETQPTMIAASVDALADATELALSGQTATRVLVFDHHRQVDAHRAAVESARERLAGSAVVETLAEAIARGDVPRGASAGSAPGTDVSDDSLALLIYTSGSTGAPKGAMYPRRNVATFWRKRTWFEGGYEPSITLNFMPMSHVMGRQILYGTLCNGGTAYFVAKSDLSTLFEDLALVRPTELTFVPRVWDMVFDEFQSEVDRRLVDGADRVALEAQVKAEIRNDVLGGRYTSALTGSAPISDEMKAWVEELLDMHLVEGYGSTEAGMILIDGAIRRPAVLDYKLVDVPDLGYFLTDRPHPRGELLVKTDSLFPGYYQRAEVTADVFDADGFYRTGDIMAEVGPEQFVYLDRRNNVLKLSQGEFVTVSKLEAVFGDSPLVRQIYIYGNSARAYLLAVIVPTQEALDAVPVEELKARLGDSLQEVAKAAGLQSYEIPRDFIIETTPWTLENGLLTGIRKLARPQLKKHYGELLEQIYTDLAHGQADELRSLRQSGADAPVLVTVCRAAAALLGGSASDVQPDAHFTDLGGDSLSALSFTNLLHEIFDIEVPVGVIVSPANDLQALADYVEAARKPGSSRPTFASVHGASNGQVTEVHAGDLSLDKFIDAATLAEAPRLPAANTQVRTVLLTGATGFLGRYLALEWLERMDLVDGKLICLVRAKSDTEARARLDKTFDSGDPELLAHYRALAGDHLEVLAGDKGEADLGLDRQTWQRLADTVDLIVDPAALVNHVLPYSQLFGPNALGTAELLRLALTSKIKPYSYTSTIGVADQIPPSAFTEDADIRVISATRAVDDSYANGYSNSKWAGEVLLREAHDLCGLPVAVFRCDMILADTTWAGQLNVPDMFTRMILSLAATGIAPGSFYELAADGARQRAHYDGLPVEFIAEAISTLGAQSQDGFHTYHVMNPYDDGIGLDEFVDWLNESGCPIQRIADYGDWLQRFETALRALPDRQRHSSLLPLLHNYRQPERPVRGSIAPTDRFRAAVQEAKIGPDKDIPHVGAPIIVKYVSDLRLLGLL

SEQ ID NO: 20 - protein, 1178 aa, Mycobacterium abscessus
MTETISTAAVPTTDLEEQVKRRIEQVVSNDPQLAALLPEDSVTEAVNEPDLPLVEVIRRLLEGYGDRPALGQRAFEFVTGDDGATVIALKPEYTTVSYRELWERAEAIAAAWHEQGIRDGDFVAQLGFTSTDFASLDVAGLRLGTVSVPLQTGASLQQRNAILEETRPAVFAASIEYLDAAVDSVLATPSVRLLSVFDYHAEVDSQREALEAVRARLESAGRTIVVEALAEALARGRDLPAAPLPSADPDALRLLIYTSGSTGTPKGAMYPQWLVANLWQKKWLTDDVIPSIGVNFMPMSHLAGRLTLMGTLSGGGTAYYIASSDLSTFFEDIALIRPSEVLFVPRVVEMVFQRFQAELDRSLAPGESNSEIAERIKVRIREQDFGGRVLSAGSGSAPLSPEMTEFMESLLQVPLRDGYGSTEAGGVWRDGVLQRPPVTDYKLVDVPELGYFTTDSPHPRGELRLKSETMFPGYYKRPETTADVFDDEGYYKTGDVVAELGPDHLKYLDRVKNVLKLAQGEFVAVSKLEAAYTGSPLVRQIFVYGNSERSFLLAVVVPTPEVLERYADSPDALKPLIQDSLQQVAKDAELQSYEIPRDFIVETVPFTVESGLLSDARKLLRPKLKDHYGERLEALYAELAESQNERLRQLAREAATRPVLETVTDAAAALLGASSSDLAPDVRFIDLGGDSLSALSYSELLRDIFEVDVPVGVINSVANDLAAIARHIEAQRTGAATQPTFASVHGKDATVITAGELTLDKFLDESLLKAAKDVQPATADVKTVLVTGGNGWLGRWLVLDWLERLAPNGGKVYALIRGADAEAARARLDAVYESGDPKLSAHYRQLAQQSLEVIAGDFGDQDLGLSQEVWQKLAKDVDLIVHSGALVNHVLPYSQLFGPNVAGTAEIIKLAISERLKPVTYLSTVGIADQIPVTEFEEDSDVRVMSAERQINDGYANGYGNSKWAGEVLLREAHDLAGLPVRVFRSDMILAHSDYHGQLNVTDVFTRSIQSLLLTGVAPASFYELDADGNRQRAHYDGVPGDFTAASITAIGGVNVVDGYRSFDVFNPHHDGVSMDTFVDWLIDAGYKIARIDDYDQWLARFELALKGLPEQQRQQSVLPLLKMYEKPQPAIDGSALPTAEFSRAVHEAKVGDSGEIPHVTKELILKYASDIQLLGLV

SEQ ID NO: 21 - protein, 1193 aa, Mycobacterium smegmatis
MHQLTVTGMNICEVQRLFPRMTSDVHDATDGVTETALDDEQSTRRIAELYATDPEFAAAAPLPAVVDAAHKPGLRLAEILQTLFTGYGDRPALGYRARELATDEGGRTVTRLLPRFDTLTYAQVWSRVQAVAAALRHNFAQPIYPGDAVATIGFASPDYLTLDLVCAYLGLVSVPLQHNAPVSRLAPILAEVEPRILTVSAEYLDLAVESVRDVNSVSQLVVFDHHPEVDDHRDALARAREQLAGKGIAVTTLDAIADEGAGLPAEPIYTADHDQRLAMILYTSGSTGAPKGAMYTEAMVARLWTMSFITGDPTPVINVNFMPLNHLGGRIPISTAVQNGGTSYFVPESDMSTLFEDLALVRPTELGLVPRVADMLYQHHLATVDRLVTQGADELTAEKQAGAELREQVLGGRVITGFVSTAPLAAEMRAFLDITLGAHIVDGYGLTETGAVTRDGVIVRPPVIDYKLIDVPELGYFSTDKPYPRGELLVRSQTLTPGYYKRPEVTASVFDRDGYYHTGDVMAETAPDHLVYVDRRNNVLKLAQGEFVAVANLEAVFSGAALVRQIFVYGNSERSFLLAVVVPTPEALEQYDPAALKAALADSLQRTARDAELQSYEVPADFIVETEPFSAANGLLSGVGKLLRPNLKDRYGQRLEQMYADIAATQANQLRELRRAAATQPVIDTLTQAAATILGTGSEVASDAHFTDLGGDSLSALTLSNLLSDFFGFEVPVGTIVNPATNLAQLAQHIEAQRTAGDRRPSFTTVHGADATEIRASELTLDKFIDAETLRAAPGLPKVTTEPRTVLLSGANGWLGRFLTLQWLERLAPVGGTLITIVRGRDDAAARARLTQAYDTDPELSRRFAELADRHLRVVAGDIGDPNLGLTPEIWHRLAAEVDLVVHPAALVNHVLPYRQLFGPNVVGTAEVIKLALTERIKPVTYLSTVSVAMGIPDFEEDGDIRTVSPVRPLDGGYANGYGNSKWAGEVLLREAHDLCGLPVATFRSDMILAHPRYRGQVNVPDMFTRLLLSLLITGVAPRSFYIGDGERPRAHYPGLTVDFVAEAVTTLGAQQREGYVSYDVMNPHDDGISLDVFVDWLIRAGHPIDRVDDYDDWVRRFETALTALPEKRRAQTVLPLLHAFRAPQAPLRGAPEPTEVFHAAVRTAKVGPGDIPHLDEALIDKYIRDLREFGLI

SEQ ID NO: 22 - protein, 1178 aa, Mycobacterium smegmatis
MTETISTAAVPTTDLEEQVKRRIEQVVSNDPQLAALLPEDSVTEAVNEPDLPLVEVIRRLLEGYGDRPALGQRAFEFVTGDDGATVIALKPEYTTVSYRELWERAEAIAAAWHEQGIRDGDFVAQLGFTSTDFASLDVAGLRLGTVSVPLQTGASLQQRNAILEETRPAVFAASIEYLDAAVDSVLATPSVRLLSVFDYHAEVDSQREALEAVRARLESAGRTIVVEALAEALARGRDLPAAPLPSADPDALRLLIYTSGSTGTPKGAMYPQWLVANLWQKKRLTDDVIPSIGVNFMPMSHLMGRLTLMGTLSGGGTAYYIASSDLSTFFEDIALIRPSEVLFVPRVVEMVFQRFQAELDRSLAPGESNSEIAERIKVRIREQDFGGRVLSAGSGSAPLSPEMTEFMESLLQVPLRDGYGSTEAGGVWRDGVLQRPPVTDYKLVDVPELGYFTTDSPHPRGELRLKSETMFPGYYKRPETTADVFDDEGYYKTGDVVAELGPDHLKYLDRVKNVLKLAQGEFVAVSKLEAAYTGSPLVRQIFVYGNSERSFLLAVVVPTPEVLERYADSPDALKPLIQDSLQQVAKDAELQSYEIPRDFIVETVPFTVESGLLSDARKLLRPKLKDHYGERLEALYAELAESQNERLRQLAREAATRPVLETVTDAAAALLGASSSDLAPDVRFIDLGGDSLSALSYSELLRDIFEVDVPVGVINSVANDLAAIARHIEAQRTGAATQPTFASVHGKDATVITAGELTLDKFLDESLLKAAKDVQPATADVKTVLVTGGNGWLGRWLVLDWLERLAPNGGKVYALIRGADAEAARARLDAVYESGDPKLSAHYRQLAQQSLEVIAGDFGDQDLGLSQEVWQKLAKDVDLIVHSGALVNHVLPYSQLFGPNVAGTAEIIKLAISERLKPVTYLSTVGIADQIPVTEFEEDSDVRVMSAERQINDGYANGYGNSKWAGEVLLREAHDLAGLPVRVFRSDMILAHSDYHGQLNVTDVFTRSIQSLLLTGVAPASFYELDADGNRQRAHYDGVPGDFTAASITAIGGVNVVDGYRSFDVFNPHHDGVSMDTFVDWLIDAGYKIARIDDYDQWLARFELALKGLPEQQRQQSVLPLLKMYEKPQPAIDGSALPTAEFSRAVHEAKVGDSGEIPHVTKELILKYASDIQLLGLV

SEQ ID NO: 23 - protein, 224 aa, Bacillus subtilis
MKIYGIYMDRPLSQEENERFMTFISPEKREKCRRFYHKEDAHRTLLGDVLVRSVISRQYQLDKSDIRFSTQEYGKPCIPDLPDAHFNISHSGRWVIGAFDSQPIGIDIEKTKPISLEIAKRFFSKTEYSDLLAKDKDEQTDYFYHLWSMKESFIKQEGKGLSLPLDSFSVRLHQDGQVSIELPDSHSPCYIKTYEVDPGYKMAVCAAHPDFPEDITMVSYEELL

SEQ ID NO: 24 - protein, 222 aa, Nocardia iowensis
MIETILPAGVESAELLEYPEDLKAHPAEEHLIAKSVEKRRRDFIGARHCARLALAELGEPPVAIGKGERGAPIWPRGVVGSLTHCDGYRAAAVAHKMRFRSIGIDAEPHATLPEGVLDSVSLPPEREWLKTTDSALHLDRLLFCAKEATYKAWWPLTARWLGFEEAHITFEIEDGSADSGNGTFHSELLVPGQTNDGGTPLLSFDGRWLIADGFILTAIAYA

SEQ ID NO: 25 - protein, 272 aa, Saccharomyces cerevisiae
MVKTTEVVSEVSKVAGVRPWAGIFVVEIQEDILADEFTFEALMRTLPLASQARILNKKSFHDRCSNLCSQLLQLFGCSIVTGLNFQELKFDKGSFGKPFLDNNRFLPFSMTIGEQYVAMFLVKCVSTDEYQDVGIDIASPCNYGGREELELFKEVFSEREFNGLLKASDPCTIFTYLWSLKESYTKFTGTGLNTDLSLIDFGAISFFPAEGASMCITLDEVPLIFHSQWFNNEIVTICMPKSISDKINTNRPKLYNISLSTLIDYFIENDGL

SEQ ID NO: 26 - protein, 209 aa, Escherichia coli
MVDMKTTHTSLPFAGHTLHFVEFDPANFCEQDLLWLPHYAQLQHAGRKRKTEHLAGRIAAVYALREYGYKCVPAIGELRQPVWPAEVYGSISHCGTTALAVVSRQPIGIDIEEIFSVQTARELTDNIITPAEHERLADCGLAFSLALTLAFSAKESAFKASEIQTDAGFLDYQIISWNKQQVIIHRENEMFAVHWQIKEKIVITLCQHD

SEQ ID NO: 27 - protein, 468 aa, Escherichia coli
MIREPPEHILNRLPSSASALACSAHALNLIEKRTLDHEEMKALNREVIEYFKEHVNPGFLEYRKSVTAGGDYGAVEWQAGSLNTLVDTQGQEFIDCLGGFGIFNVGHRNPVVVSAVQNQLAKQPLHSQELLDPLRAMLAKTLAALTPGKLKYSFFCNSGTESVEAALKLAKAYQSPRGKFTFIATSGAFHGKSLGALSATAKSTFRKPFMPLLPGFRHVPFGNIEAMRTALNECKKTGDDVAAVILEPIQGEGGVILPPPGYLTAVRKLCDEFGALMILDEVQTGMGRTGKMFACEHENVQPDILCLAKALGGGVMPIGATIATEEVFSVLFDNPFLHTTTFGGNPLACAAALATINVLLEQNLPAQAEQKGDMLLDGFRQLAREYPDLVQEARGKGMLMAIEFVDNEIGYNFASEMFRQRVLVAGTLNNAKTIRIEPPLTLTIEQCELVIKAARKALAAMRVSVEEA

SEQ ID NO: 28 - protein, 456 aa, Pseudomonas aeruginosa
MNSQITNAKTREWQALSRDHHLPPFTDYKQLNEKGARIITKAEGVYIWDSEGNKILDAMAGLWCVNVGYGREELVQAATRQMRELPFYNLFFQTAHPPVVELAKAIADVAPEGMNHVFFTGSGSEANDTVLRMVRHYWATKGQPQKKVVIGRWNGYHGSTVAGVSLGGMKALHEQGDFPIPGIVHIAQPYWYGEGGDMSPDEFGVWAAEQLEKKILEVGEENVAAFIAEPIQGAGGVIVPPDTYWPKIREILAKYDILFIADEVICGFGRTGEWFGSQYYGNAPDLMPIAKGLTSGYIPMGGVVVRDEIVEVLNQGGEFYHGFTYSGHPVAAAVALENIRILREEKIIEKVKAETAPYLQKRWQELADHPLVGEARGVGMVAALELVKNKKTRERFTDKGVGMLCREHCFRNGLIMRAVGDTMIISPPLVIDPSQIDELITLARKCLDQTAAAVLA

SEQ ID NO: 29 - protein, 426 aa, Escherichia coli
MNSNKELMQRRSQAIPRGVGQIHPIFADRAENCRVWDVEGREYLDFAGGIAVLNTGHLHPKVVAAVEAQLKKLSHTCFQVLAYEPYLELCEIMNQKVPGDFAKKTLLVTTGSEAVENAVKIARAATKRSGTIAFSGAYHGRTHYTLALTGKVNPYSAGMGLMPGHVYRALYPCPLHGISEDDAIASIHRIFKNDAAPEDIAAIVIEPVQGEGGFYASSPAFMQRLRALCDEHGIMLIADEVQSGAGRTGTLFAMEQMGVAPDLTTFAKSIAGGFPLAGVTGRAEVMDAVAPGGLGGTYAGNPIACVAALEVLKVFEQENLLQKANDLGQKLKDGLLAIAEKHPEIGDVRGLGAMIAIELFEDGDHNKPDAKLTAEIVARARDKGLILLSCGPYYNVLRILVPLTIEDAQIRQGLEIISQCFDEAKQ

SEQ ID NO: 30 - protein, 421 aa, Escherichia coli
MSNNEFHQRRLSATPRGVGVMCNFFAQSAENATLKDVEGNEYIDFAAGIAVLNTGHRHPDLVAAVEQQLQQFTHTAYQIVPYESYVTLAEKINALAPVSGQAKTAFFTTGAEAVENAVKIARAHTGRPGVIAFSGGFHGRTYMTMALTGKVAPYKIGFGPFPGSVYHVPYPSDLHGISTQDSLDAIERLFKSDIEAKQVAAIIFEPVQGEGGFNVAPKELVAAIRRLCDEHGIVMIADEVQSGFARTGKLFAMDHYADKPDLMTMAKSLAGGMPLSGVVGNANIMDAPAPGGLGGTYAGNPLAVAAAHAVLNIIDKESLCERANQLGQRLKNTLIDAKESVPAIAAVRGLGSMIAVEFNDPQTGEPSAAIAQKIQQRALAQGLLLLTCGAYGNVIRFLYPLTIPDAQFDAAMKILQDALSD

SEQ ID NO: 31 - protein, 464 aa, Ruegeria pomeroyi
MATITNHMPTAELQALDAAHHLHPFSANNALGEEGTRVITRARGVWLNDSEGEEILDAMAGLWCVNIGYGRDELAEVAARQMRELPYYNTFFKTTHVPAIALAQKLAELAPGDLNHVFFAGGGSEANDTNIRMVRTYWQNKGQPEKTVIISRKNAYHGSTVASSALGGMAGMHAQSGLIPDVHHINQPNWWAEGGDMDPEEFGLARARELEEAILELGENRVAAFIAEPVQGAGGVIVAPDSYWPEIQRICDKYDILLIADEVICGFGRTGNWFGTQTMGIRPHIMTIAKGLSSGYAPIGGSIVCDEVAHVIGKDEFNHGYTYSGHPVAAAVALENLRILEEENILDHVRNVAAPYLKEKWEALTDHPLVGEAKIVGMMASIALTPNKASRAKFASEPGTIGYICRERCFANNLIMRHVGDRMIISPPLVITPAEIDEMFVRIRKSLDEAQAEIEKQGLMKSAA

SEQ ID NO: 32 - protein, 339 aa, Escherichia coli
MSMIKSYAAKEAGGELEVYEYDPGELRPQDVEVQVDYCGICHSDLSMIDNEWGFSQYPLVAGHEVIGRVVALGSAAQDKGLQVGQRVGIGWTARSCGHCDACISGNQINCEQGAVPTIMNRGGFAEKLRADWQWVIPLPENIDIESAGPLLCGGITVFKPLLMHHITATSRVGVIGIGGLGHIAIKLLHAMGCEVTAFSSNPAKEQEVLAMGADKVVNSRDPQALKALAGQFDLIINTVNVSLDWQPYFEALTYGGNFHTVGAVLTPLSVPAFTLIAGDRSVSGSATGTPYELRKLMRFAARSKVAPTTELFPMSKINDAIQHVRDGKARYRVVLKADF

SEQ ID NO: 33 - DNA, 1206 bp, Escherichia coli
atgcgtgaagcctttatttgtgacggaattcgtacgccaattggtcgctacggcggggcattatcaagtgttcgggctgatgatctggctgctatccctttgcgggaactgctggtgcgaaacccgcgtctcgatgcggagtgtatcgatgatgtgatcctcggctgtgctaatcaggcgggagaagataaccgtaacgtagcccggatggcgactttactggcggggctgccgcagagtgtttccggcacaaccattaaccgcttgtgtggttccgggctggacgcactggggtttgccgcacgggcgattaaagcgggcgatggcgatttgctgatcgccggtggcgtggagtcaatgtcacgggcaccgtttgttatgggcaaggcagccagtgcattttctcgtcaggctgagatgttcgataccactattggctggcgatttgtgaacccgctcatggctcagcaatttggaactgacagcatgccggaaacggcagagaatgtagctgaactgttaaaaatctcacgagaagatcaagatagttttgcgctacgcagtcagcaacgtacggcaaaagcgcaatcctcaggcattctggctgaggagattgttccggttgtgttgaaaaacaagaaaggtgttgtaacagaaatacaacatgatgagcatctgcgcccggaaacgacgctggaacagttacgtgggttaaaagcaccatttcgtgccaatggggtgattaccgcaggcaatgcttccggggtgaatgacggagccgctgcgttgattattgccagtgaacagatggcagcagcgcaaggactgacaccgcgggcgcgtatcgtagccatggcaaccgccggggtggaaccgcgcctgatggggcttggtccggtgcctgcaactcgccgggtgctggaacgcgcagggctgagtattcacgatatggacgtgattgaactgaacgaagcgttcgcggcccaggcgttgggtgtactacgcgaattggggctgcctgatgatgccccacatgttaaccccaacggaggcgctatcgccttaggccatccgttgggaatgagtggtgcccgcctggcactggctgccagccatgagctgcatcggcgtaacggtcgttacgcattgtgcaccatgtgcatcggtgtcggtcagggcatcgccatgattctggagcgtgtttga

SEQ ID NO: 34 - DNA, 35 bp, Artificial Sequence
  paaJ(Ec) pRSFDuet cloning fw
ataaggagatataccatgcgtgaagcctttatttg

SEQ ID NO: 35 - DNA, 35 bp, Artificial Sequence
  paaJ(Ec) pRSFDuet cloning rv
tgcggccgcaagctttcaaacacgctccagaatca

SEQ ID NO: 36 - DNA, 25 bp, Artificial Sequence
  pRSFDuet MCS1 Backbone Fw
aagcttgcggccgcataatgcttaa

SEQ ID NO: 37 - DNA, 20 bp, Artificial Sequence
  pRSFDuet MCS1 Backbone Rv
catggtatatctccttatta

SEQ ID NO: 38 - DNA, 1428 bp, Escherichia coli
atgatgataaatgtgcaaactgtggcagtgattgggagcggcaccatgggggcaggcattgctgaagttgctgccagtcatggacaccaggttttactgtatgacatttctgctgaagcgctgacccgcgcaatcgacgggatacacgcgcggctaaattcacgcgtgacgcggggaaaactgactgctgaaacctgtgaacgcacattgaaacgcctgatcccggtgaccgatattcacgcgctggcagctgcggacctggtcattgaagcggcgtctgaacgtctggaagtcaaaaaagcgctctttgcacagctggcggaagtttgcccgccacaaacgctattgaccactaacacttcgtcaatctctataaccgcgattgctgcggagataaaaaatcctgaacgtgttgcggggctgcatttttttaacccggcaccggtgatgaagttggtggaggtggtcagtgggctggcaacggcggcggaagttgttgagcagttgtgtgaactaacgttgagttggggtaagcagcctgtgcgctgtcattcgactcctggatttatcgttaaccgtgttgcgcgtccttattattccgaggcctggcgggcactggaagagcaggttgctgcaccagaagtgattgacgctgcacttcgcgatggcgctggtttcccgatggggccgctggaattaaccgatctgattggtcaggacgtcaattttgctgtcacctgttcggtgtttaacgctttctggcaggagcgtcgttttttaccttcgctggtgcaacaggaactggtgattggtggacggttgggcaagaaaagtgggctgggcgtgtacgactggcgcgcggaacgtgaggcagttgttggcctggaagcggtaagcgacagttttagcccaatgaaagtagaaaagaaaagtgacggtgtcacggaaattgacgatgttttattgattgagacacaaggcgagacggcacaggcgctggcaatacgactggcacgcccggtggtagtgatcgataaaatggcgggcaaggtggtgaccattgctgctgcagcggtgaacccggactcagcgacccgcaaggccatttattacctgcaacagcagggcaaaacagtgctgcaaattgcagattacccaggaatgctgatttggcgaacggtagcaatgatcatcaatgaagcccttgatgcgcttcaaaaaggcgtggcctctgaacaggatatcgataccgccatgcgtcttggggtgaattatccatatggcccacttgcctggggagcgcaacttggctggcagcgaatattaaggctccttgaaaatctacagcatcactatggcgaagaacgctatcgcccatgttcattgctgcgccaacgggcgcttctggagagcggttatgagtcataa

SEQ ID NO: 39 - DNA, 35 bp, Artificial Sequence
  paaH(Ec) pRSFDuet cloning fw
ggagatatacatatgatgataaatgtgcaaactgt

SEQ ID NO: 40 - DNA, 35 bp, Artificial Sequence
  paaH(Ec) pRSFDuet cloning rv
agactcgagggtaccttatgactcataaccgctct

SEQ ID NO: 41 - DNA, 25 bp, Artificial Sequence
  pRSFDuet MCS2 Backbone Fw
ggtaccctcgagtctggtaaagaaa

SEQ ID NO: 42 - DNA, 20 bp, Artificial Sequence
  pRSFDuet MCS2 Backbone Rv
catatgtatatctccttctt

SEQ ID NO: 43 - DNA, 768 bp, Escherichia coli
atgagcgaactgatcgtcagccgtcagcaacgagtattgttgctgacccttaaccgtcccgccgcacgtaatgcgctaaataatgccctgctgatgcaactggtaaatgaactggaagctgcggctaccgataccagcatttcggtctgtgtgattaccggtaatgcacgcttttttgccgctggggccgatctcaacgaaatggcagaaaaagatctcgcggccaccttaaacgatacacgtccgcagctatgggcgcgattgcaggcctttaataaaccacttatcgcagccgtcaatggttacgcgcttggggcgggttgcgaactggcattgttgtgcgatgtggtggttgccggagagaacgcgcgttttgggttgccggaaatcactctcggcatcatgcctggcgcaggcggaacgcaacgtttaatccgtagtgtcggtaaatcgttagccagcaaaatggtgctgagcggagaaagtatcaccgctcagcaagcacagcaggccgggctggttagcgacgtcttccccagcgatttaaccctcgaatacgccttacagctggcatcgaaaatggcacgtcactcgccgctggccttacaagcggcaaagcaagcgctgcgccagtcgcaggaagtggctttgcaagccggacttgcccaggagcgacagttattcaccttgctggcggcaacagaagatcgtcatgaaggcatctccgctttcttacaaaaacgcacgcccgactttaaaggacgctaa

SEQ ID NO: 44 - DNA, 35 bp, Artificial Sequence
  paaF(Ec) pETDuet cloning fw
aggagatataccatgagcgaactgatcgtcagccg

SEQ ID NO: 45 - DNA, 35 bp, Artificial Sequence
  paaF(Ec) pETDuet cloning rv
tgcggccgcaagcttttagcgtcctttaaagtcgg

SEQ ID NO: 46 - DNA, 24 bp, Artificial Sequence
  primer
ttaacgtcctgcataggtgggttt

SEQ ID NO: 47 - DNA, 35 bp, Artificial Sequence
  paaF(L3)opt pETDuet cloning fw
agaaggagatataccatgcagaccattgaaaatga

SEQ ID NO: 48 - DNA, 35 bp, Artificial Sequence
  paaF(L3)opt pETDuet cloning rv
tgcggccgcaagcttttaacgaccggcataggtcg

SEQ ID NO: 49 - DNA, 25 bp, Artificial Sequence
  pETDuet MCS1 Backbone fw
aagcttgcggccgcataatgcttaa

SEQ ID NO: 50 - DNA, 25 bp, Artificial Sequence
  pETDuet MCS1 Backbone rv
catggtatatctccttcttaaagtt

SEQ ID NO: 51 - DNA, 1155 bp, Acinetobacter baylyi
atgattcgtgatgaaggtatgctgcaacagctgctgagcaccattcgtgattttgttaaaaatgaactgattccgcgtgaacatgaagtggcagaaaaagattgtattcccgaagatattattcagcagatgcgtgaactgggtctgtttggtctgaccattccggaagaatatggtggtctgggtattaccatggaagaagaagttaacgttgcatttgaactgggccagaccagtccggcatttcgtagcctgattggcaccaataatggtattggtagcagcggtctgattattgatggcaccgaagaacagaaacagaaatatctgcctcgttatgcaagcggtgaaattattggtagtttttgtctgaccgaaccggaagcaggtagtgatgcagcaagcctgaaaaccaccgcagttaaagatggtgatttctatattctgaacggcaccaaacgctttattaccaatgcaccgcatgcagcaacctttaccgttatggcacgtaccaatccggcaattaaaggtgccggtggtattagcgcatttctggttgaagcaaatacaccgggtattacgctgggtaaaattgatcagaaaatgggtcagaaaggtagccatacctgtgatgtgatttttgaaaattgtcgtgttccggcaagcgcactgattggtggtgttgaaggtgttggctttaaaaccgcaatgaaagttctggataaaggtcgtctgcatattggtgcatatagcgttggtgttgcagaacgtatgctgaatgatgcactgcattatgccgttgaacgtaaacagtttggtcagccgattgcaaattttcagctgattcaggcaatgctggcagatagcaaagcagaaatttatgcagccaaatgcatggttctggatgcagcacgtcgtcgtgatgagggtcagaatattagcaccgaagcaagctgtgcaaaaatgtttgcaaccgaaatgtgtggtcgtgttgccgatcgttgtgttcagattcatggtggtgcaggttatattagcgaatacagcattgaacgcttctatcgtgatgtgcgtctgtttcgcctgtatgaaggtacaacccaggtgcagcagattattatcgccaaaaacatgatcaaagaggtgaccagctaa

SEQ ID NO: 52 - DNA, 35 bp, Artificial Sequence
  dcaA(Ab)opt pETDuet cloning fw
gaaggagatatacatatgattcgtgatgaaggtat

SEQ ID NO: 53 - DNA, 35 bp, Artificial Sequence
  dcaA(Ab)opt pETDuet cloning rv
tggcagcagcctaggttagctggtcacctctttga

SEQ ID NO: 54 - DNA, 1095 bp, Candida tropicalis
atgattaccgcacaggcagttctgtatacccagcatggtgaaccgaaagatgtgctgtttacccagagctttgaaatcgatgatgataatctggcaccgaacgaagttattgttaaaaccctgggtagtccggttaatccgagcgatattaatcagattcagggtgtttatccgagcaaaccggcaaaaaccaccggttttggcaccaccgaaccggcagcaccgtgtggtaatgaaggtctgtttgaagttattaaagtgggcagcaatgttagcagcctggaagccggtgattgggttattccgagccatgtgaattttggtacatggcgtacccatgcactgggcaatgatgatgattttatcaaactgccgaatccggcacagagcaaagcaaatggtaaaccgaatggcctgaccattaatcagggtgcaaccattagcgttaatccgctgaccgcatatctgatgctgacccattatgttaaactgacaccgggtaaagattggtttattcagaatggtggcaccagcgcagttggtaaatatgcaagccagattggtaaactgctgaactttaatagcattagcgtgattcgtgatcgtccgaatctggatgaagttgttgcaagcctgaaagaactgggtgcgacccaggttattaccgaagatcagaataatagccgtgaatttggtccgaccattaaagaatggattaaacagagcggtggtgaagcaaaactggcactgaattgtgttggtggtaaaagcagcaccggtattgcacgtaaactgaataataacggtctgatgttaacctatggtggcatgagctttcagccggttaccattccgaccagcctgtatatctttaaaaactttaccagtgccggtttttgggttaccgagctgctgaaaaataacaaagaactgaaaaccagcacgctgaaccagattattgcatggtatgaagagggtaaactgaccgatgcaaaaagcattgaaaccctgtatgatggcaccaaaccgctgcatgaactgtatcaggatggtgttgcaaatagcaaagatggcaaacagctgatcacctactaa

SEQ ID NO: 55 - DNA, 35 bp, Artificial Sequence
  ter(Ct)opt N22AAcut  pETDuet cloning fw
gaaggagatatacatatgattaccgcacaggcagt

SEQ ID NO: 56 - DNA, 35 bp, Artificial Sequence
  ter(Ct)opt N22AAcut pETDuet cloning rv
tggcagcagcctaggttagtaggtgatcagctgtt

SEQ ID NO: 57 - DNA, 1167 bp, Candida auris
atgtttgttccaaccgttgctgggaaacgctttctgaccaatcagctgcgcaaaagtccgcagttcacccgtatgctgacttcacacgcggtgattttcagctctcatggggaacccaaagacgttctgaaaacgcatacgtacgaaatcgatgagaacaacatcaaacccaacgagattgtcctgaaaaccttgggtgctccggtcaatccatcggacattaaccaggtgcagggtgtatatcctagccaaccggagaaaacgacccaactgggaacttcggaaccgtcagccgttggtggcaatgaagggctctttgagatcatcaaaattggcagtgatgtgaaaggctttcaagttggtgattgggccattccgacctcggtcaactttggtacgtggcgtagtcatgcgctgtgcgaagaaggcaaaatgatgaaagtcccgaacccggaacagtctaaacaggccggtaagaaacagggcttaaccatcaatcaaggtgcgaccttaagcgtgaatccgcttacagcctaccttatgctcacacactacgtgaaactcacaccgggtaaggactggtttatccagaacggtggcaatagcgcagtcggaaaatttgcgagccaaattgggaaattactggggattcatagcatttccgtggttcgcgatcgtcctgaaattgaagaactgaagaaagagctgaaggaagtatgtggtgcgactcaggtaatcaccgaagagcagaacaactccaaggacttcggccctcaggtgaagcagtgggtgaaagaaactggcggcgagatcaaactggcgctgaattgcgtaggtggcaaaagcagtgcaggcgttgcacggaaactcgctcccaacggactgatgctgacatatggcggcatgtcatttcaaccggtaaccttgccaacgagcttgcacattttcaagaatgtgacgtctgcgggcttctgggtgacggaactgctgaaatctgatccgaacctgaaacgcgaaaccgttgacaaaattgtcgagtggtatacctcaggcgaattacttgatgcgccatcgaaagaaaatcagtggggtgatcaagatctggcacaagtgttcattgatgccgtcgccaactccaaatccggaaaacagttggtgaagttttaa

SEQ ID NO: 58 - DNA, 1143 bp, Kluyveromyces marxianus
atgagttcatttctcagcaaacgcttcattagcacgacgcaacgtgccatgagccaattgccgaaagccaaatcgctgatctactcatcccatgatcaggacgtgagtaaaatcctgaaagtgcatacttaccagccgaaagggtcagcggaaagctcgatcctgctcaaaacgttagcctttccgatcaatccttccgacatcaaccaactggaaggggtatatccgagtaagccggaaaaggtgttggattactcaacggaagaaccgagcgctattgctggcaatgagggtctgtttgaggttgtatcggtacctagcggtgtcaagaatctgaaagctggtgaccgtgtcattccacttcaggcgaactttggcacctggtctacgtatcgcacatgcgaaagcgagaatgacttgatcaaaatcgaaggcgtagatctctataccgcagcaaccattgcggtgaatggctgtaccgcgtaccaaatggtgaatgactacattgagtgggatcctagtggcaacgattggctggttcagaacgcgggtacaagttctgtatccaaaattgtgacccagatcgctaaagacaagggcatcaaaaccctgtcggtggttcgtgatcgcgataactttgacgaagttgcggagaaactggaaaagaaatatggtgcgaccaaagtgatttctgaaagccagaacggagaacgtgagttcgggaatgaagtcttaccgaagattcttggtcccaatgcccaggttaaactcgcgttaaactctgtgggcggtaaaagctgcactaacattgcccgcaaactgagtccaaacggattaatgctgacctatggcggcatgtccaaacagccggttacactgccaactggcctgtttatcttcaatagcattcggtcgcacggtttctgggttaccgcaaattcgaaacgcgatcccgaaaacaaacggaaaactgtggatgccgtggtcaaactgtatcgcgatggcaagattatttccccgaaagaggacattcgtaccctggaatgggatgtcaacaatctgtctgatgaaggtgtccttgatttggtcaaccgcggaattgcaacgaaaggggcaaagaacatggttgtgctgaaatggtaa

SEQ ID NO: 59 - DNA, 1122 bp, Pichia kudriavzevii
atgagtctgcgttccgtgtttagcgtgagttccattcgtcggatgtcctctatcacggctcgcgcaatcgtctataacgcgcatggcgaaccgaaagataccctgaaatgccacagctacaagatcgaccttcagaatttacagcctaacgaggttgtcgtacaaactctcgcagcgccactgaacccgagtgatatcaaccagattcagggtgtttacccgtctaagcctccgctgagcattgactcactgccagaactgaaagaaccggccgctgttactggcaatgagggtgtgttcaaagtgattgccaaagggtcgaatgtaggagaactggaaacgggagactggtgtattccgtctggcgtaaactttggtacctggtgtacgcaccgcttaaccacggataagaatctgctgaaaatgccgaaaaccatctcgttaaaccaggcagcaaccattgccgtcaacccctcatcggcatatcagatgctgacgcactttgtgaaactgcaaccaggtgattggtttatccagaatggcgccaattcccaagttggtcgtgcagcgattcagattggccataaactggggtacaaatcgttgaacattgttcgcaaccgtgacaacttggatgagctggtgaaggacctggaatcgattggggcgactaaagtgattacagaagatgaaagcgcgagcaaagagtttggcgctacggttaaagagtggcttgagggcaaagagatcaaactcggtctgaattgcattggtggtccgtctgcgtcaaacttagcccgcaaattgggccatgatgctaccatcctgacgtatggcgcgatgagcaagaaaccgctctcattgccgactgggaatttcatctttaagaatctcaccgccaaaggattttggattacaggtaacatcaaacgccatccagaactgcgcatcgaaaccattaatgcggtcctgaaattcatggaagatggcacccttaaggaacctaaagtgaacgaacccaaagtcaaactgagtaccacaacaaatgaaagcttccttgaaaccgtgctggccgcgttggaagatagccaaaagggcaaacaactgttaaaattcgaataa

SEQ ID NO: 60 - DNA, 1347 bp, Thermothelomyces thermophilus
atggcgtcagtcttatcaccaaacgcagcagcacgtcatctgctgcgtcctgctacccggtctacaccgcctcgtttactgccgtccgcaatcttacaccaaagcggcaataactccacgcgcaatccgcgcattagcgatccgcagtcaattgctcaacggttaggtcgtcgctacaaatcgggcccgtacggctatacgcaggccaaaacgctggtgttttcgcgtttcggagaaccctccgatgttctgcgcctgcatacgcatagcatcagtccgacactgccggatggtgcggttctggtgcgggcactggcagctccagtaaacccggcggatgtcaacactatccaaggcacctatggtgcgcgtccagctttcagccccttactcggcactcccgaacctagtgcggttccaggcaacgaaggttgctttgaagttgtcgcagttggtccacgtgtcggcggcggtctgcgtaaaggggattgggtgattccggccaccaccggctttggcacctttcgcacacacgcgttggtggagaatgccgatcgcgctctgcttcgcgtaggaggtgacaaaggtaccgcgggtctgaccgccaaacaggtggccacggtaagcgtcaatccgtgttcggcctatcgtatgctcaaggactacgtcgatctggtggacttgagtgtgaagtcctttgctcgcggtgatggggccactggcggggcgtggtttctccagaatggcgcgaatagcggagttggtcgcgcggcgattcagctgggccgcctctggggtctgcgctcgattaacgtggttcgtgaacgcgctaccgccgaagaaaccgaagcattgaaaagcgaactgcgtgagcttggtgcgacggttgttgtgaccgaagcggaattccttgatcgctctttctcggcccgcttgaaagaagagtggacacgcggcgatcgcgaaccggtgatgctgggtttgaactgtgtaggcgggaaaagcgcgagcgccatgatcaaggccctgtctccgaaaggttgcatggtgacttatggcgggatgagtcgtcagtcattcccctttccgactggtcctcagatctttaaacgcctgcgttttgagggattctggctgagtgaatgggccaaagagaatccggcggagaaacgcaacaccattaatgagattctggagctgatgcgggaaggcaaattcaaagagtctccgttcaaagaagtggaatggaactgggacacggaagaaaaggtactgaaagacgcaattcaaggcacccttgaagggttcaagtccgggaaaggattatttgtctttggcgacacgtaa

SEQ ID NO: 61 - DNA, 1332 bp, Thermothielavioides terrestris
atggccagcgccttgaatcctcgccatctgccgctgcgcttagccttacgtcctcgcttgccactgctgccatccacgagctctaccaccacaaccacaaccccaccctcgtgtctgccgattccgacctctattcgtctgcctccccgtcgtcacaaatcagggccgtatggttacacgcttgcgaaaaccttagtgtttagtcgctttggtgaaccccgcgatgtactgtcgcttcatacccacagcattagccccgcactgccggatggggcggctctgttacgcgctcttgcagcgccggtcaatccggcggacgtaaacaccgtccaagggacctatggcgccaaaccggcgtttgagcgtctgctgggtactccggaaccggctgcagtaccgggcaatgagggttgcttcgaagtcgttgccattggtggaggtgccggtggtggcggtggtcttaagaaaggtgactgggttattcctgcacagagtggcttcggcaccttccgcacacatgcgttggtggaaggcgcagaacgcaaactgattcgtgtgggaggcgccaaagggcgtgaaggtctgcgtgctgcgcaagttgcgacggtgtctgtgaatccatgtagcgcatatcggatgctccgtgattacgtagacttagtggacctgagcgtgcagtcatttgctcgcggtgatggcgcaaccggcggcgcgtggttcgtgcagaacggagccaacagtggcgttggtcgtgcggctattcaactgggacgtctgtggggcttgcgttcgatcaacgtggttcgggaacgtgcgactccggaagaaaccgcggccttaaaacgcgaactcgccgagttgggtgcaacggtagtcgttacggaatccgaattcctcgatcgctcgtttgctgaccggctgcgcgatgagtggactcgcggcggccgcgaaccggtgatgctcggtctgaactgcgttggcgggaaatctgccgcagccatggtcaaagcgctgagtccacgcggatgcatggtcacatacggcggtatgagccgccagtccttcccgtttccgactggccagcagatctttaagcgcctgcgctttgagggcttttggctgtcagagtgggcgaaagagaatcctgcggcgaaacgggataccatcaacgagattctggaattgatgcgtgaaggcaaattcaaggaagcaccgctccaagaagttgaatggaactgggatacggaagaatccgtgctgaaagacacgatccaggggactctggaggggtttcgcccaggcaaaagcatcttcgtctttaaggatacgtaa

SEQ ID NO: 62 - DNA, 1320 bp, Chaetomium thermophilum
atggctagcatcctgtcccctcattctgctctccgtttgggaggaatctccacgctgtcacgtcagaccctgctgcgtacctctcgtgtgaccttaacccagttaccgaaaaccgctccgcagttaccgcaacgtcggcataaaagtgcgccttacggctatacccagtccaaaacgctggtgtttccgcgtttcggggagccgattgacgttctgtcgttacacactcactcgattagcccgacccttcccgatactgcggtgctgcttcgcacgctggcggcgcccattaatcctgcggacgtcaacacgattcaggggacctatggcgcaaagccgacgttcagcaacttactgggcaccgcagagcctgcagcagttccggggaatgaaggtgtatttgaggtcgtttcggttggctcggaaattgcaaaacgtggcgtgttcaagaaaggtgattgggtcattccgagcagtagcggctttggcacttttcgcacccatgtactggttgaagaagcggagcagaaactgtggcgcattggcggcgagaaaggcaccgaaggtttaacgccagtacaggtcgcaacggtttcggtgaatccgtgttctgcgtatcgcatgctgcgtgactatgtggatctggtgggcgtgagcgtacgcatgtaccaggaaggtgggtcagatgtccgtggtggagcgtggttcctgcaaaatggcgccaactcaggtgttggacgcgctgccattcaactcgggcgtttgtggggtttgcgctcaatcaacgtggtacgggagcgcgcgactgccgaagaaacagaagccctgaagaaagagctgtacgatcttggggccactgtggtggtgaccgaatccgaattcctggatcgcagttttacacagcgcctgaatgaggaatggacacggggaggtaaagagccattgctgcttgccctgaactgcgtgggtggcaaaagtgcccaacagattgttcgcgctctgtctccgaaaggcactatggtcacgtatggcggtatgagccgccaaagctttccgtttccgacgggtccacagatctttaaacgtctgcgctttgaaggtttctggctctccgaatgggccaaagaaaaccccgcagaaaagaagaaatgcgtagatgagatcatcgaactgatgcgcgaaggcaaattcaaagaagcgccagtccaggaaattcgctgggattgggaaaccgaagaaaaggtcttgaaagaggcggttcaaggcacactcgaaggctttcgcagtggtaaaggtgtgtttatcttcggtgacacctaa

SEQ ID NO: 63 - DNA, 1269 bp, Podospora anserina
atggcagctccgcgtctgacctctaaagccttacgcttaccgacgagcaaactcttgcgtccagcgctgacaactgctacgcctcgcgcagccccaaccttgacccagaaacgtcatctgactggtccatatggctaccaccagagcaaagcgctgaccttctccagctttggcgaaccgattgacgtgctctcactgcatacgcactcgattagtccgacattaccctcaggtagtgtcttagtgcgtactctcgcggcaccggtaaacccggcagacgttaacaccattcaagggacctacggatccaagccgccctttacgacgctgttgggtacggcccaaccgtcggcggttccgggcaatgaagcgtgctttgaggtgctgtctgtgggccaaggggtgaaagggctcgaaaagggcgattgggtcattccagccaagactgggttcggcacctttcggactcatgcccttgtggaagaagctgaggggaaactgatgcgtgtagaacgcgaaggcttgacgccggttcaggtagccaccgttagcgtcaacccttgttcggcgtatcgcatgctgaaagactacgtggatctggttggcctgtccatgcgctggtatcgcgaaggtaaagatgtgagcggtggcgcctggttcctgcagaatggcgcgaactctggagttggccgtgcggccgtgcaatttggccgtttgtggggtttacgcagcatcaacgttgtacgcgaacgtgaaacacctgaagaaaccgaaaagttaaaagaagaactgacgggtttgggtgcgaacgtcgtcctgaccgagcaggaatttcttgatcgctcttttcgcgatcggctgggtgagctgacgaaacgcggtaaagaacccctgctgcttggtatgaattgtgtgggcggaaaatccgcatcagcggtagtcaaagctctctcgccaaaaggctgcatggtcacctatggcggtatgagtcgtcagagcttcccgtttcctactggtccgcagatcttcaagcgtctgcgcttcgaaggcttctggctttcagagtggggtaaagagaatccggaagggaagaagaaaatgatcgaagatattctgaacctgatgcgcgaagggaaattcaaagaaagcccggttcaagaggtggagtggaattgggaaaccgaggagaaaaccctgaaagaggcagttcagggaacactgggtggctttcgcagtggcaaaggcgtgtttgtgtttggagaaacctaa

SEQ ID NO: 64 - DNA, 1275 bp, Purpureocillium lilacinum
atggcgagtagtcgcctgctcggaccaccactgcgcctcccaagctcgggattcagccgcccggttgctgccctgaattgtcgtgcggcagcactgcccttgcatctgccacgtacagcggtccggtatcgttcggggccttacggttacactcaggcgaaggcccttgtgtacagcaagaacggcgaaccggcagatgtgctgaagttacacacgcacagtatttccccttcaattccgtccacctccgttctggtacgctgcctggccgctccgattaacccggctgatgtcaacacgattcaggggacctatggcagcaaacaaccgctcacgagcttaattgggaccagtgaaccctccgcagttccgggcaatgaaggcgtctttgaagttctctcagccggttccccgagcagcgagctgaagaagggagattgggtgatccctgccgcatctcagattggcacatggcgcacccatgcggtgtttggggctgacgagctcttgaaagtcgacaaagagggtctgacgccgactcaagtttctcttgtgtcggttaacccgtgtacggcgtatcgcatcctgcggagctatggtccctcagctggcgtgaaagcggcgttaggcatgcgcccgttagaggtgggtagtggacagtggtttatccagaatggcgcgaattctggcgttggccgtgcagccattcagtttggcaaactgtggggcttgcgctcgatcaacgtcattcgcgaccgtgacaccgtcgaagccacagacgcactgaaacaggagttgcgggatttgggcgcggatgtcgtagttgctgaatctgagttcctgtctcgtggttggaaagaccaactggcggaaattacccgcaaagggcgtgaacaggtagggcttggcctgaattgcgtgggtggcaaatcagccacggcacttgcgcgtagcctgggtgaaggtgccactctggtaagctatggtggtatggcgaaacaaccggtggcgttacctgtcggtctgttgatcttcaaagatatccgcttcgttggcttttggctgtcgaaatggaaccagcaggatgtggtgggtcgtcgccatatggtagcagacatcctgggactgatgcgtgacggtaaattccgcgatgccccggtggatgaagtgaaatgggattgggataccgatgaagcgaccctgcgtggggctgcccaacgcggcttagaaggttttcgccaaggtaaaggcgtatacgtgtttggcgatacctaa

SEQ ID NO: 65 - DNA, 1218 bp, Pyrenophora teres
atggcgtctaaactgatctcgcctagtccgcgcctcgcacagagctgtttacgccgcactcgtaatttggccccggtgactgcgcgctttccccaacgccgctacatctctgcctatgggtatgaacaggcaaaagctctgacgtttaccgaatacggggatccatctgcggtgctgagcttgcacagccactccatctcgccgcctcatagcaactatatgaccctgcgcttcctggcgagcccgatcaatccagcagacattaaccaaattcagggcgtttatccgtccaaacccacttttacgacgtcgctgggtactccgaacccaattgccgtcgctggcaatgaaggcgtggcggaaattattgcgctgggtgaaggtgttaagaaagaaggcttcaagaaaggcgattgggtctttatgaaaggcccgggctttggcacatggcgtacccatgccagtgcaactaccaacgatgtcgtcaagctgaatgaccagatgcgggaaggtatcacggccattcaagcgggcaccgtttcaattaatccgtgcaccgcttatcgtatgcttcgggattttaccaccctgagcgaaggagattggtttatccagaatggcgccaattcaggcgtgggtcgtgcagcaattcagctgggtcgcaaatggggatacaaatccattaacattattcgcagtcgtgaggataagaacaaagaagaggcgatgaagaaagagctgcataacctcggggccgatgtggtaattacggatgcagagttacaagcgcaagggatcaaagaccaggccaaagagtggacaaacggtggacgtagccctattcgccttgcgttaaactgcgtgaatggcaaagctgctaccgcgatggcgaaactgctgtcgagttcagcccatttcgtaacctatggtgcgatgtccaagcagccgttgaccatcccagccagcatgcttattttcaaagatatccactttcatggtttctgggtgtctcgctgggcagaagaacacccggaagagaaacagaaaacggttgcggatgtcctcgacatgacacgtaagggagagttcaaagacatgccggttgatgaaatcaaatgggaatgggaaacaaaaggggaggaactggttgctaaagtgaaagacacgttagaaggttaccgtgacggtaaaggcatcttcgtatttggcaaaacctaa

SEQ ID NO: 66 - DNA, 35 bp, Artificial Sequence
  ter(caur) pETDuet cloning fw
gaaggagatatacatatgtttgttccaaccgttgc

SEQ ID NO: 67 - DNA, 35 bp, Artificial Sequence
  ter(caur) pETDuet cloning rv
tggcagcagcctaggttaaaacttcaccaactgtt

SEQ ID NO: 68 - DNA, 35 bp, Artificial Sequence
  ter(kmx) pETDuet cloning fw
gaaggagatatacatatgagttcatttctcagcaa

SEQ ID NO: 69 - DNA, 35 bp, Artificial Sequence
  ter(kmx) pETDuet rv
tggcagcagcctaggttaccatttcagcacaacca

SEQ ID NO: 70 - DNA, 35 bp, Artificial Sequence
  ter(pkz) pETDuet cloning fw
gaaggagatatacatatgagtctgcgttccgtgtt

SEQ ID NO: 71 - DNA, 35 bp, Artificial Sequence
  ter(pkz) pETDuet cloning rv
tggcagcagcctaggttattcgaattttaacagtt

SEQ ID NO: 72 - DNA, 35 bp, Artificial Sequence
  ter(mtm) pETDuet cloning fw
gaaggagatatacatatggcgtcagtcttatcacc

SEQ ID NO: 73 - DNA, 35 bp, Artificial Sequence
  ter(mtm) pETDuet cloning rv
tggcagcagcctaggttacgtgtcgccaaagacaa

SEQ ID NO: 74 - DNA, 35 bp, Artificial Sequence
  ter(ttt) pETDuet cloning fw
gaaggagatatacatatggccagcgccttgaatcc

SEQ ID NO: 75 - DNA, 35 bp, Artificial Sequence
  ter(ttt) pETDuet Ecloning rv
tggcagcagcctaggttacgtatccttaaagacga

SEQ ID NO: 76 - DNA, 35 bp, Artificial Sequence
  ter(cthr) pETDuet cloning fw
gaaggagatatacatatggctagcatcctgtcccc

SEQ ID NO: 77 - DNA, 35 bp, Artificial Sequence
  ter(cthr) pETDuet cloning rv
tggcagcagcctaggttaggtgtcaccgaagataa

SEQ ID NO: 78 - DNA, 35 bp, Artificial Sequence
  ter(pan) pETDuet cloning fw
gaaggagatatacatatggcagctccgcgtctgac

SEQ ID NO: 79 - DNA, 35 bp, Artificial Sequence
  ter(pan) pETDuet cloning rv
tggcagcagcctaggttaggtttctccaaacacaa

SEQ ID NO: 80 - DNA, 35 bp, Artificial Sequence
  ter(plj) pETDuet cloning fw
gaaggagatatacatatggcgagtagtcgcctgct

SEQ ID NO: 81 - DNA, 35 bp, Artificial Sequence
  ter(plj) pETDuet cloning rv
tggcagcagcctaggttaggtatcgccaaacacgt

SEQ ID NO: 82 - DNA, 35 bp, Artificial Sequence
  ter(pte) pETDuet Ecloning fw
gaaggagatatacatatggcgtctaaactgatctc

SEQ ID NO: 83 - DNA, 35 bp, Artificial Sequence
  ter(pte) pETDuet cloning rv
tggcagcagcctaggttaggttttgccaaatacga

SEQ ID NO: 84 - DNA, 25 bp, Artificial Sequence
  pETDuet MCS2 Backbone Fw
cctaggctgctgccaccgctgagca

SEQ ID NO: 85 - DNA, 25 bp, Artificial Sequence
  pETDuet MCS2  Backbone Rv
catatgtatatctccttcttatact

SEQ ID NO: 86 - DNA, 3537 bp, Artificial Sequence
  Mab4714opt W283RA303A
atgaccgaaaccattagcaccgcagcagttccgaccaccgatctggaagaacaggttaaacgtcgtattgaacaggttgttagcaatgatccgcagctggcagccctgctgccggaagatagcgttaccgaagcagttaatgaaccggatctgccgctggttgaagttattcgtcgtctgctggaaggttatggtgatcgtccggcactgggtcagcgtgcatttgaatttgttaccggtgatgatggtgcaaccgttattgcactgaaaccggaatacaccaccgttagctatcgtgaactgtgggaacgtgccgaagcaattgcagcagcatggcatgaacagggtattcgtgatggtgattttgttgcacagctgggttttaccagcaccgattttgcaagcctggatgttgcaggtctgcgtctgggtacagttagcgttccgctgcagaccggtgccagcctgcagcagcgtaatgcaatcctggaagaaacccgtccggcagtttttgcagcaagcattgaatatctggatgcagcagttgatagcgttctggcaaccccgagcgtgcgtctgctgagcgtttttgattatcatgccgaagtggatagccagcgtgaagcactggaagcagttcgtgcacgtctggaaagcgcaggtcgtaccattgttgttgaagccctggccgaagcgctggcacgtggtcgtgatctgccagcagcaccgctgccgagtgccgatccggatgcactgcgcctgctgatttataccagcggtagcaccggtacaccgaaaggtgccatgtatccgcagtggctggttgcaaatctgtggcagaaaaaaaggctgaccgatgatgttattccgagcattggtgtgaattttatgccgatgagccatctgatgggtcgtctgaccctgatgggcaccctgagcggtggtggcaccgcctattatatcgcaagcagcgatctgagcaccttttttgaagatattgccctgattcgtccgagcgaagttctgtttgttccgcgtgttgtggaaatggtttttcagcgttttcaggcagaactggatcgtagcctggctccgggtgaaagcaatagcgaaattgcagaacgtattaaagtgcgtattcgcgaacaggattttggtggtcgtgtgctgagcgcaggtagcggtagtgcaccgctgagtccggaaatgaccgaatttatggaaagcctgctgcaagtgccgctgcgtgatggttatggtagtaccgaagccggtggtgtttggcgtgatggcgttctgcagcgtccgcctgttaccgattataaactggttgatgtgccggaactgggttattttaccaccgatagtccgcatccgcgtggtgaactgcgtctgaaaagcgaaaccatgtttccgggttattacaaacgtccggaaaccaccgcagatgtttttgatgatgaaggctattacaaaacgggtgatgtggttgctgaactgggtcctgatcatctgaaatacctggatcgtgttaaaaacgttctgaaactggcacagggtgaatttgtggcagttagcaaactggaagccgcatataccggtagtccgctggttcgtcagatttttgtttatggtaatagcgaacgtagctttctgctggccgttgttgttccgacaccggaagttctggaacgttatgcagatagtccggatgcgctgaaaccgctgattcaggatagtctgcagcaggttgcaaaagatgcagaactgcagagctatgaaattccgcgtgattttattgttgaaaccgttccgtttaccgttgaaagcggactgctgagtgatgcacgtaaactgttacgtccgaaactgaaagatcattatggtgaacgcctggaagccctgtatgccgaactggcagaaagccagaatgaacgtctgcgtcagctggcacgcgaagcagcaacacgtccggttctggaaaccgttaccgatgccgcagccgcactgctgggtgcaagcagctccgatctggcaccagatgttcgttttattgatttaggtggtgatagcctgagcgcactgagctatagcgagctgctgcgcgatatttttgaagttgatgttccggttggtgtgattaatagcgttgcaaatgatctggcagcaattgcccgtcatattgaagcacagcgtacaggtgcagcaacccagccgacctttgcaagcgttcatggtaaagatgccaccgttattaccgcaggcgaactgaccctggataaatttctggatgaaagtctgctgaaagcagccaaagatgttcagcctgcgacagcagatgttaaaaccgtgctggtgaccggtggtaatggctggttaggtcgttggctggttctggattggctggaacgtctggcaccgaatggtggtaaagtttatgcactgattcgtggtgcagatgcggaagcagcacgcgcacgcctggatgccgtttatgaaagcggtgatcctaaactgagtgcacattatcgtcaactggcccagcagagcctggaagttattgcaggcgattttggcgatcaggatctgggtctgagccaagaagtttggcagaaactggcgaaagatgttgatctgattgttcatagcggtgccctggttaatcatgttctgccgtatagccagctgtttggtccgaatgttgccggtacagcagaaattatcaaactggcaattagcgaacgcctgaaacctgttacctatctgagtaccgttggtattgcagatcagattccggttaccgaatttgaagaggatagtgatgttcgcgttatgagcgcagaacgtcagattaatgatggctatgcaaatggctatggcaatagcaaatgggctggtgaagttctgctgcgtgaagcccatgatttagccggtctgccggttcgtgtttttcgtagcgatatgattctggcacatagcgattatcacggtcagctgaatgtgaccgatgtttttacccgtagcattcagagtctgctgctgacaggtgttgcaccggcaagcttttatgaactggatgcggatggtaatcgccagcgtgcccattatgatggtgttccaggtgattttaccgcagccagcattaccgcaattggtggtgttaatgttgtggatggttatcgcagctttgatgtgtttaatccgcatcacgatggtgttagcatggatacctttgttgattggctgattgatgccggttacaaaattgcacgcatcgatgattatgatcagtggttagcacgttttgaactggccctgaaaggcctgcctgaacagcagcgtcagcagagcgttctgccactgctgaaaatgtatgaaaaaccgcagcctgcaattgatggtagcgcactgccgaccgcagaatttagccgtgcagttcatgaagcaaaagtgggtgatagtggtgaaatcccgcatgttaccaaagaactgattctgaaatatgccagcgatattcagctgctgggtttagtttaa

SEQ ID NO: 87 - DNA, 35 bp, Artificial Sequence
  pACYCDuet Mab4714opt cloning fw
gaaggagatatacatatgaccgaaaccattagcac

SEQ ID NO: 88 - DNA, 35 bp, Artificial Sequence
  pACYCDuet Mab4714opt cloning rv
gtggcagcagcctagttaaactaaacccagcagct

SEQ ID NO: 89 - DNA, 669 bp, Nocardia iowensis
atgatcgagacaattttgcctgctggtgtcgagtcggctgagctgctggagtatccggaggacctgaaggcgcatccggcggaggagcatctcatcgcgaagtcggtggagaagcggcgccgggacttcatcggggccaggcattgtgcccggctggcgctggctgagctcggcgagccgccggtggcgatcggcaaaggggagcggggtgcgccgatctggccgcgcggcgtcgtcggcagcctcacccattgcgacggatatcgggccgcggcggtggcgcacaagatgcgcttccgttcgatcggcatcgatgccgagccgcacgcgacgctgcccgaaggcgtgctggattcggtcagcctgccgccggagcgggagtggttgaagaccaccgattccgcactgcacctggaccgtttactgttctgcgccaaggaagccacctacaaggcgtggtggccgctgaccgcgcgctggctcggcttcgaggaagcgcacatcaccttcgagatcgaagacggctccgccgattccggcaacggcacctttcacagcgagctgctggtgccgggacagacgaatgacggtgggacgccgctgctttcgttcgacggccggtggctgatcgccgacgggttcatcctcaccgcgatcgcgtacgcctga

SEQ ID NO: 90 - DNA, 35 bp, Artificial Sequence
  Npt cloning fw
tttaaggagttcgatatgatcgagacaattttgcc

SEQ ID NO: 91 - DNA, 35 bp, Artificial Sequence
  Npt rv
ggtggcagcagcctagtcaggcgtacgcgatcgcg

SEQ ID NO: 92 - DNA, 20 bp, Artificial Sequence
  Mab4714opt_pACYCDuet Npt insertion backbone Fw
ctaggctgctgccaccgctg

SEQ ID NO: 93 - DNA, 45 bp, Artificial Sequence
  Mab4714opt_pACYCDuet Npt insertion backbone Rv
atcgaactccttaaatttatttaaactaaacccagcagctgaata

SEQ ID NO: 94 - DNA, 1020 bp, Escherichia coli
atgtcgatgataaaaagctatgccgcaaaagaagcgggcggcgaactggaagtttatgagtacgatcccggtgagctgaggccacaagatgttgaagtgcaggtggattactgcgggatctgccattccgatctgtcgatgatcgataacgaatggggattttcacaatatccgctggttgccgggcatgaggtgattgggcgcgtggtggcactcgggagcgccgcgcaggataaaggtttgcaggtcggtcagcgtgtcgggattggctggacggcgcgtagctgtggtcactgcgacgcctgtattagcggtaatcagatcaactgcgagcaaggtgcggtgccgacgattatgaatcgcggtggctttgccgagaagttgcgtgcggactggcaatgggtgattccactgccagaaaatattgatatcgagtccgccgggccgctgttgtgcggcggtatcacggtctttaaaccactgttgatgcaccatatcactgctaccagccgcgttggggtaattggtattggcgggctggggcatatcgctataaaacttctgcacgcaatgggatgcgaggtgacagcctttagttctaatccggcgaaagagcaggaagtgctggcgatgggtgccgataaagtggtgaatagccgcgatccgcaggcactgaaagcactggcggggcagtttgatctcattatcaacaccgtcaacgtcagcctcgactggcagccctattttgaggcgctgacctatggcggtaatttccatacggtcggtgcggttctcacgccgctgtctgttccggcctttacgttaattgcgggcgatcgcagcgtctctggttctgctaccggcacgccttatgagctgcgtaagctgatgcgttttgccgcccgcagcaaggttgcgccgaccaccgaactgttcccgatgtcgaaaattaacgacgccatccagcatgtgcgcgacggtaaggcgcgttaccgcgtggtgttgaaagccgatttttga

SEQ ID NO: 95 - DNA, 35 bp, Artificial Sequence
  Ahr cloning fw
ataaggagatataccatgtcgatgataaaaagcta

SEQ ID NO: 96 - DNA, 35 bp, Artificial Sequence
  Ahr cloning rv
atgcggccgcaagcttcaaaaatcggctttcaaca

SEQ ID NO: 97 - DNA, 35 bp, Artificial Sequence
  pACYCDuet MCS1 Backbone Fw
catggtatatctccttattaaagttaaacaaaatt

SEQ ID NO: 98 - DNA, 30 bp, Artificial Sequence
  pACYCDuet MCS1 Backbone Rv
agcttgcggccgcataatgcttaagtcgaa

SEQ ID NO: 99 - DNA, 35 bp, Artificial Sequence
  atoB-del-f1
ttgttgaataaatcggcactcggtatcgcttacct

SEQ ID NO: 100 - DNA, 35 bp, Artificial Sequence
  atoB-del-r1
tatcgcatgcagatcggctggtggtcaacggtgcc

SEQ ID NO: 101 - DNA, 35 bp, Artificial Sequence
  sucD-del-f1
ttgttgaataaatcggagcgcgacctggcgttgat

SEQ ID NO: 102 - DNA, 35 bp, Artificial Sequence
  sucD-del-r1
tatcgcatgcagatcacgatatttttcagttaacc

SEQ ID NO: 103 - DNA, 35 bp, Artificial Sequence
  ldhA-del-f1
ttgttgaataaatcgtttatcgatattgatccagg

SEQ ID NO: 104 - DNA, 35 bp, Artificial Sequence
  ldhA-del-r1
tatcgcatgcagatctgtgtgcattacccaacggc

SEQ ID NO: 105 - DNA, 35 bp, Artificial Sequence
  adhE-del-f1
ttgttgaataaatcgctgccgctgtctgataactg

SEQ ID NO: 106 - DNA, 35 bp, Artificial Sequence
  adhE-del-r1
tatcgcatgcagatctcgatatacccgtactttgt

SEQ ID NO: 107 - DNA, 35 bp, Artificial Sequence
  dkgA-HA-flag-f
ttgttgaataaatcgtctgtttgccgagaatacgc

SEQ ID NO: 108 - DNA, 35 bp, Artificial Sequence
  dkgA-HA-flag-r
tatcgcatgcagatccgaccattttccgccaccat

SEQ ID NO: 109 - DNA, 35 bp, Artificial Sequence
  yahK-del-f1
ttgttgaataaatcgatattcgtcctaacgaacag

SEQ ID NO: 110 - DNA, 35 bp, Artificial Sequence
  yahK-del-r1
tatcgcatgcagatctttttgattttcaagtatgt

SEQ ID NO: 111 - DNA, 35 bp, Artificial Sequence
  ahr-del-f1
ttgttgaataaatcgctcataacggtactgcaaac

SEQ ID NO: 112 - DNA, 35 bp, Artificial Sequence
  ahr-del-r1
tatcgcatgcagatctcgcagcaggtaagatgatt

SEQ ID NO: 113 - DNA, 35 bp, Artificial Sequence
  pflB-del-f1
ttgttgaataaatcgatcacctggggtcagttggc

SEQ ID NO: 114 - DNA, 35 bp, Artificial Sequence
  pflB-del-r1
tatcgcatgcagatccgtcgttcatctgtttgaga

SEQ ID NO: 115 - DNA, 33 bp, Artificial Sequence
  pHAK-v-fw
gatctgcatgcgatatctctagaacgcgtaagc

SEQ ID NO: 116 - DNA, 28 bp, Artificial Sequence
  pHAK-v-rev3
cgatttattcaacaaagccgccgtcccg

SEQ ID NO: 117 - DNA, 20 bp, Artificial Sequence
  atoB-del-f2-2
cgatggtgattgaacggttg

SEQ ID NO: 118 - DNA, 20 bp, Artificial Sequence
  atoB-del-r2-2
gcactgacgatgacacaatt

SEQ ID NO: 119 - DNA, 20 bp, Artificial Sequence
  sucD-del-f2-2
gaaattcgctgctctggaag

SEQ ID NO: 120 - DNA, 23 bp, Artificial Sequence
  sucD-del-r2-2
cctggcagataaccttggtgttt

SEQ ID NO: 121 - DNA, 20 bp, Artificial Sequence
  ldhA-del-f2-2
tggtttaatcttgccgctcc

SEQ ID NO: 122 - DNA, 22 bp, Artificial Sequence
  ldhA-del-r2-2
gtgctataaacggcgagtttca

SEQ ID NO: 123 - DNA, 26 bp, Artificial Sequence
  adhE-del-f2
tcagtagcgctgtctggcaatataaa

SEQ ID NO: 124 - DNA, 30 bp, Artificial Sequence
  adhE-del-r2
aatgctctcctgataatgttaaactttttt

SEQ ID NO: 125 - DNA, 25 bp, Artificial Sequence
  yqhD-del-f2
catgcaaattctcccggtggcggta

SEQ ID NO: 126 - DNA, 24 bp, Artificial Sequence
  yqhD-del-r2
ccaatatgagggcagagaacgatc

SEQ ID NO: 127 - DNA, 20 bp, Artificial Sequence
  yahK-del-f2-2
tcgcacactaacagactgaa

SEQ ID NO: 128 - DNA, 20 bp, Artificial Sequence
  yahK-del-r2
tgtgtttactcctgattagc

SEQ ID NO: 129 - DNA, 24 bp, Artificial Sequence
  ahr-del-f2-2
cgtggtgttgaaagccgattattg

SEQ ID NO: 130 - DNA, 23 bp, Artificial Sequence
  ahr-del-r2-2
cataaacttccagttctccgccc

SEQ ID NO: 131 - DNA, 32 bp, Artificial Sequence
  pflB-del-f2
ttagatttgactgaaatcgtacagtaaaaagc

SEQ ID NO: 132 - DNA, 27 bp, Artificial Sequence
  pflB-del-r2
gtaacacctaccttcttaagtggattt

SEQ ID NO: 133 - DNA, 186 bp, Artificial Sequence
  promoter region
gcagctgctgcagctcgagagatctctcaagcccaaaggaagagtgaggcgagtcagtcgcgtaatgcttaggcacaggattgatttgtcgcaatgattgacacgattccgcttgacgctgcgtaaggtttgtgtataattacaggcaaccttttattcactaacaaatagctggtggaagatatc

SEQ ID NO: 134 - DNA, 16 bp, Artificial Sequence
  linker region
agaaggagatatacat

SEQ ID NO: 135 - DNA, 162 bp, Artificial Sequence
  terminator region
ggtaccctcgagtctggtaaagaaaccgctgctgcgaaatttgaacgccagcacatggactcgtctactagcgcagcttaattaacctaggctgctgccaccgctgagcaataactagcataaccccttggggcctctaaacgggtcttgaggggttttttg

SEQ ID NO: 136 - DNA, 186 bp, Artificial Sequence; identical to SEQ ID NO: 133
  promoter region

SEQ ID NO: 137 - DNA, 30 bp, Artificial Sequence
  linker region
aagcttgcggccgcagaaggagatatacat

SEQ ID NO: 138 - DNA, 76 bp, Artificial Sequence
  terminator region
ctaggctgctgccaccgctgagcaataactagcataaccccttggggcctctaaacgggtcttgaggggttttttg

SEQ ID NO: 139 - DNA, 186 bp, Artificial Sequence; identical to SEQ ID NO: 133
  promoter region

SEQ ID NO: 140 - DNA, 20 bp, Artificial Sequence
  linker region
ataaatttaaggagttcgat

SEQ ID NO: 141 - DNA, 76 bp, Artificial Sequence; identical to SEQ ID NO: 138
  terminator region

SEQ ID NO: 142 - DNA, 23 bp, Artificial Sequence
  atoB check Fw2
aagcagctaccgaaagatgcccc

SEQ ID NO: 143 - DNA, 30 bp, Artificial Sequence
  atoB check Rv2
ggcagatgatcaaaatatctcagcgcagat

SEQ ID NO: 144 - DNA, 20 bp, Artificial Sequence
  sucD-check-f
gggtctggaaggtaaactgg

SEQ ID NO: 145 - DNA, 23 bp, Artificial Sequence
  sucD-check-r
cgtcaaagaagagcgggtcaatt

SEQ ID NO: 146 - DNA, 21 bp, Artificial Sequence
  ldhA-check-f
agaggttaatgcgagagagag

SEQ ID NO: 147 - DNA, 20 bp, Artificial Sequence
  ldhA-check-r
ctggatggtacggcgattgg

SEQ ID NO: 148 - DNA, 26 bp, Artificial Sequence
  adhE-check-f
tcgacatcgctatcgtcaccaccagg

SEQ ID NO: 149 - DNA, 26 bp, Artificial Sequence
  adhE-check-r
cgcgtataggtttgtcatcgcctgca

SEQ ID NO: 150 - DNA, 25 bp, Artificial Sequence
  dkgA-check-Fw
tattctcaatccgtttcagcacgcg

SEQ ID NO: 151 - DNA, 24 bp, Artificial Sequence
  dkgA-check-Rv
ggattattggccgtcttgaaggtg

SEQ ID NO: 152 - DNA, 25 bp, Artificial Sequence
  yahK-check-f2
agctgaccatcagtcacgcctttgc

SEQ ID NO: 153 - DNA, 28 bp, Artificial Sequence
  yahK-check-r2
cgtccagaacagagagcaataacatcac

SEQ ID NO: 154 - DNA, 20 bp, Artificial Sequence
  ahr-check-f
tccgctagtgtgatttcagg

SEQ ID NO: 155 - DNA, 23 bp, Artificial Sequence
  ahr-check-r
gaaattattatgccgccaggcgt

SEQ ID NO: 156 - DNA, 25 bp, Artificial Sequence
  pflB-check-f
ctgattctttgtgttgtctgcggag

SEQ ID NO: 157 - DNA, 25 bp, Artificial Sequence
  pflB-check-r
cagatatttagcgaactccagcgtg

SEQ ID NO: 158 - protein, 468 aa, Artificial Sequence
  YgjG(m)
MIREPPEHILNRLPSSASALACSAHALNLIEKRTLDHKEMKALNREVIEYYKEHVNPGFLEYRKSVTAGGDYGAVEWQAGSLNTLVDTQGQEFIDCLGGFGIFNVGHRNPVVVSAVQNQLAKQPLHSQELLDPLRAMLAKTLAALTPGKLKYSFFCNSGTESVEAALKLAKAYQSPRGKFTFIATSGAFHGKSLGALSATAKSTFRKPFMPLLPGFRHVPFGNIEAMRRALNECKKTGDDVAAVILEPIQGEGGVILPPPGYLTAVRKLCDEFGALMILDEVQTGMGRTGKMFACEHENVQPDILCLAKALGGGVMPIGATIATEEVFSVLFDNPFLHTTTFGGNPLACAAALATINVLLEQNLPAQAEQKGDMLLDGFRQLAREYPDLVQEARGKGMLMAIEFVDNEIGYNFASEMFRQRVLVAGTLNNAKTIRIEPPLTLTIEQCELVIKAARKALAAMRVSVEEA

SEQ ID NO: 159 - DNA, 1407 bp, Artificial Sequence
  ygjG (m)
atgatacgcgagcctccggagcatattttgaacaggttaccttcgagcgcatcggctttagcgtgcagcgcccacgccctgaatctcattgagaagcgaacgctggatcataaggagatgaaagcacttaaccgagaggtgattgaatactacaaagagcatgtcaatccggggtttttagagtatcgcaaatctgttaccgccggcggggattacggagccgtagagtggcaagcgggaagtttaaatacgcttgtcgacacccagggccaggagtttatcgactgcctgggaggttttggaattttcaacgtggggcaccgtaatccagttgtggtttccgccgtacagaatcaacttgcgaaacaaccgctgcacagccaggaactgctcgatccgttacgggcgatgttggcgaaaacccttgctgcgctaacgcccggtaaactgaaatacagcttcttctgtaatagcggcaccgagtccgttgaagcagcgctgaagctggcgaaagcttaccagtcaccgcgcggcaagtttacttttattgccaccagcggcgcgttccacggtaaatcacttggcgcgctgtcggccacggcgaaatcgaccttccgcaaaccgtttatgccgttactgccgggcttccgtcatgtgccgtttggcaatatcgaagccatgcgcagggctcttaacgagtgcaaaaaaaccggtgatgatgtggctgcggtgatcctcgaaccgattcagggtgaaggtggcgtaattctgccgccgccgggctatctcaccgccgtacgtaagctatgcgatgagttcggcgcactgatgatcctcgatgaagtacaaacgggcatggggcgcacgggcaagatgttcgcctgcgagcatgagaacgtacagccggatatcctctgccttgccaaagcgctcggcggcggcgtgatgccgattggcgcgaccatcgccactgaagaggtgttttcagttctgttcgacaacccattcctgcataccaccacctttggcggcaacccgctggcctgtgcggcggcgctggcgaccatcaatgtgttgctggagcagaacttaccggctcaggctgagcaaaaaggcgatatgttgctggacggtttccgtcaactggcgcgggaatatcccgatctggtacaggaagcgcgtggtaaagggatgttgatggcgattgagtttgttgataacgaaatcggctataactttgccagcgagatgttccgccagcgcgtactggtggccggaacgctcaataacgccaaaacgatccgcattgaaccgccactgacactgaccattgaacagtgtgaactggtgatcaaagcggcgcgtaaggcgctggcggccatgcgagtaagtgtcgaagaagcgtaa

SEQ ID NO: 160 - DNA, 35 bp, Artificial Sequence
  primer
ataaggagatataccatgatacgcgagcctccgga

SEQ ID NO: 161 - DNA, 35 bp, Artificial Sequence
  primer
atgcggccgcaagctttacgcttcttcgacactta

SEQ ID NO: 162 - DNA, 20 bp, Artificial Sequence
  primer
atgattcgcgaccaggaaac

SEQ ID NO: 163 - DNA, 21 bp, Artificial Sequence
  primer
tcaaacttggacgtcccgaat

SEQ ID NO: 164 - DNA, 25 bp, Artificial Sequence
  primer for paaJ
atgcttgacgcctatctctatgctg

SEQ ID NO: 165 - DNA, 23 bp, Artificial Sequence
  primer for paaJ
ttacatgcgttcgatgactacgg

SEQ ID NO: 166 - DNA, 22 bp, Artificial Sequence
  primer for paaH
atgaacactgacatccagaccc

SEQ ID NO: 167 - DNA, 19 bp, Artificial Sequence
  primer for paaH
tcagttgtcaggggtcagc

SEQ ID NO: 168 - DNA, 22 bp, Artificial Sequence
  primer for paaF
atgcaaaccatcgaaaacgaag

SEQ ID NO: 169 - DNA, 24 bp, Artificial Sequence
  primer for paaF
ttaacgtcctgcataggtgggttt

SEQ ID NO: 170 - DNA, 20 bp, Artificial Sequence
  primer for mmgC
atgattcgcgaccaggaaac

SEQ ID NO: 171 - DNA, 21 bp, Artificial Sequence
  primer for mmgC
tcaaacttggacgtcccgaat

SEQ ID NO: 172 - protein, 401 aa, Escherichia coli; identical to SEQ ID NO: 1

SEQ ID NO: 173 - protein, 475 aa, Escherichia coli
MMINVQTVAVIGSGTMGAGIAEVAASHGHQVLLYDISAEALTRAIDGIHARLNSRVTRGKLTAETCERTLKRLIPVTDIHALAAADLVIEAASERLEVKKALFAQLAEVCPPQTLLTTNTSSISITAIAAEIKNPERVAGLHFFNPAPVMKLVEVVSGLATAAEVVEQLCELTLSWGKQPVRCHSTPGFIVNRVARPYYSEAWRALEEQVAAPEVIDAALRDGAGFPMGPLELTDLIGQDVNFAVTCSVFNAFWQERRFLPSLVQQELVIGGRLGKKSGLGVYDWRAEREAVVGLEAVSDSFSPMKVEKKSDGVTEIDDVLLIETQGETAQALAIRLARPVVVIDKMAGKVVTIAAAAVNPDSATRKAIYYLQQQGKTVLQIADYPGMLIWRTVAMIINEALDALQKGVASEQDIDTAMRLGVNYPYGPLVWGAQLGWQRILRLLENLQHHYGEERYRPCSLLRQRALLESGYES

SEQ ID NO: 174 - protein, 255 aa, Escherichia coli; identical to SEQ ID NO: 3

SEQ ID NO: 175 - protein, 259 aa, Unknown
  crt(Ck)
MEFKNIILEKDGNVASITLNRPKALNALNAATLKEIDAAINDIAEDDNVYAVIITGSGKAFVAGADIAEMKDLTAVEGRKFSVLGNKIFRKLENLEKPVIAAINGFALGGGCELSLSCDIRIASSKAKFGQPEVGLGITPGFGGTQRLARAIGVGMAKELIYTGKVINAEEALRIGLVNKVVEPDKLLEEAKALVDAIIVNAPIAVRMCKAAINQGLQCDIDTGVAYEAEVFGECFATEDRVEGMTAFVEKRDKAFKNK

SEQ ID NO: 176 - protein, 276 aa, Unknown
  ch(Pp)
MSKYEGRWTTVKVELEAGIAWVTLNRPEKRNAMSPTLNREMVDVLETLEQDADAGVLVLTGAGESWTAGMDLKEYFREVDAGPEILQEKIRREASQWQWKLLRLYAKPTIAMVNGWCFGGGFSPLVACDLAICANEATFGLSEINWGIPPGNLVSKAMADTVGHRQSLYYIMTGKTFDGRKAAEMGLVNDSVPLAELRETTRELALNLLEKNPVVLRAAKNGFKRCRELTWEQNEDYLYAKLDQSRLLDTTGGREQGMKQFLDDKSIKPGLQAYKR

SEQ ID NO: 177 - protein, 384 aa, Unknown; identical to SEQ ID NO: 5
  dcaA(Ab)

SEQ ID NO: 178 - protein, 385 aa, Unknown
  Tfu1647
MSDFDLYRPTEEHEALREAIRSVAEDKIAPHAADVDEQSRFPQEAYEALRASDFHAPHVAEEYGGVGADALATCIVIEEIARVCASSSLIPAVNKLGSMPLILSGSDEVKQRYLPELASGEAMFSYGLSEREAGSDTASMRTRAVRDGDDWILNGQKSWITNAGISKYYTVMAVTDPDGPRGRNISAFVVHIDDPGFSFGEPERKLGIKGSPTRELIFDNVRIPGDRLVGKVGEGLRTALRTLDHTRVTIGAQAVGIAQGALDYALGYVKERKQFGKAIADFQGIQFMLADMAMKLEAARQMVYVAAAKSERDDADLSFYGAAAKCFASDVAMEITTDAVQLLGGYGYTRDYPVERMMRDAKITQIYEGTNQIQRVVMARQLLKK

SEQ ID NO: 179 - protein, 290 aa, Unknown
  tesB(Ab)
MNTLTQELVELLSLEKLEENLYRGMSRNLVGKRVFGGQVLGQALRAASYTTDRPAHSLHAYFLYGGDVNAPIIYEVDPLRDGKSFVSRQVRAIQHGRTIFSAMVSFASPEEGLNYQNDMPDYPAPEQLKSEAELKLGLIDFVPENVRASFMRERHIEIRPVEPVNPFQPQPQAPTNAHYIRTHDKIGKAFDQIALHQSIVAFYSDFTLMTTALKPHGLSYLSPSLQCASIDHTIYFHRPLRADEWMLYDMDATVSAGSRGLNFGRMWQNGLLVCSTVQEGLMRLREIETQ

SEQ ID NO: 180 - DNA, 1206 bp, Escherichia coli; identical to SEQ ID NO: 33

SEQ ID NO: 181 - DNA, 1428 bp, Escherichia coli
atgatgataaatgtgcaaactgtggcagtgattgggagcggcaccatgggggcaggcattgctgaagttgctgccagtcatggacaccaggttttactgtatgacatttctgctgaagcgctgacccgcgcaatcgacgggatacacgcgcggctaaattcacgcgtgacgcggggaaaactgactgctgaaacctgtgaacgcacattgaaacgcctgatcccggtgaccgatattcacgcgctggcagctgcggacctggtcattgaagcggcgtctgaacgtctggaagtcaaaaaagcgctctttgcacagctggcggaagtttgcccgccacaaacgctattgaccactaacacttcgtcaatctctataaccgcgattgctgcggagataaaaaatcctgaacgtgttgcggggctgcatttttttaacccggcaccggtgatgaagttggtggaggtggtcagtgggctggcaacggcggcggaagttgttgagcagttgtgtgaactaacgttgagttggggtaagcagcctgtgcgctgtcattcgactcctggatttatcgttaaccgtgttgcgcgtccttattattccgaggcctggcgggcactggaagagcaggttgctgcaccagaagtgattgacgctgcacttcgcgatggcgctggtttcccgatggggccgctggaattaaccgatctgattggtcaggacgtcaattttgctgtcacctgttcggtgtttaacgctttctggcaggagcgtcgttttttaccttcgctggtgcaacaggaactggtgattggtggacggttgggcaagaaaagtgggctgggcgtgtacgactggcgcgcggaacgtgaggcagttgttggcctggaagcggtaagcgacagttttagcccaatgaaagtagaaaagaaaagtgacggtgtcacggaaattgacgatgttttattgattgagacacaaggcgagacggcacaggcgctggcaatacgactggcacgcccggtggtagtgatcgataaaatggcgggcaaggtggtgaccattgctgctgcagcggtgaacccggactcagcgacccgcaaggccatttattacctgcaacagcagggcaaaacagtgctgcaaattgcagattacccaggaatgctgatttggcgaacggtagcaatgatcatcaatgaagcccttgatgcgcttcaaaaaggcgtggcctctgaacaggatatcgataccgccatgcgtcttggggtgaattatccatatggcccacttgtctggggagcgcaacttggctggcagcgaatattaaggctccttgaaaatctacagcatcactatggcgaagaacgctatcgcccatgttcattgctgcgccaacgggcgcttctggagagcggttatgagtcataa

SEQ ID NO: 182 - DNA, 768 bp, Escherichia coli; identical to SEQ ID NO: 43

SEQ ID NO: 183 - DNA, 780 bp, Unknown
  crt(Ck)
atggaattcaagaacatcatcctggaaaaagatggtaatgttgccagcattaccctgaatcgtccgaaagcactgaatgccctgaatgcagcaaccctgaaagaaattgatgcagccattaatgatatcgccgaagatgataatgtgtacgccgtgattattaccggtagcggtaaagcatttgttgccggtgcagatattgcagaaatgaaagatctgaccgcagttgaaggtcgcaaatttagcgttctgggcaataaaatctttcgcaaactggaaaatctggaaaaaccggttattgccgcaattaatggttttgcattaggtggtggttgtgaactgagcctgagctgtgatattcgtattgcaagcagcaaagcaaaatttggtcagccggaagttggtctgggtattacccctggttttggtggcacccagcgtctggcacgtgcaattggtgttggtatggcaaaagaactgatttataccggcaaagtgattaatgcagaagaagcactgcgtattggtctggttaataaagttgttgaaccggacaaactgctggaagaagcaaaagcactggttgatgccattattgttaatgcaccgattgcagttcgtatgtgtaaagcagcaattaatcagggtctgcagtgtgatattgataccggtgttgcatatgaagccgaagtttttggtgaatgttttgcaaccgaagatcgtgttgaaggtatgaccgcctttgttgaaaaacgtgataaagcctttaaaaacaaataa

SEQ ID NO: 184 - DNA, 831 bp, Unknown
  ech(Pp)
atgagcaaatatgaaggtcgttggaccaccgttaaagttgaactggaagcaggtattgcatgggttaccctgaatcgtccggaaaaacgtaatgcaatgagcccgacactgaatcgtgaaatggttgatgttctggaaaccctggaacaggatgcagatgccggtgttctggttctgaccggtgccggtgaaagctggaccgcaggtatggatctgaaagaatattttcgtgaagttgatgccggtccggaaattctgcaagaaaaaattcgtcgtgaagcaagccagtggcagtggaaactgctgcgtctgtatgcaaaaccgaccattgccatggttaatggttggtgttttggtggtggttttagtccgctggttgcatgtgatctggcaatttgtgcaaatgaagcaacctttggtctgagcgaaatcaattggggtattccgcctggtaatctggttagcaaagcaatggcagataccgttggtcatcgtcagagcctgtattatatcatgaccggtaaaacctttgatggtcgtaaagcagcagaaatgggtttagttaatgatagcgttccgctggcagaactgcgtgaaaccacacgtgaactggcactgaatctgctggaaaaaaatccggttgttctgcgtgcagcaaaaaatggttttaaacgttgtcgtgaactgacctgggaacagaatgaagattatctgtacgccaaactggatcagagccgtctgctggataccacaggtggtcgtgaacagggtatgaaacagtttctggatgacaaaagcattaaaccgggtctgcaggcatataaacgttaa

SEQ ID NO: 185 - DNA, 1155 bp, Unknown; identical to SEQ ID NO: 51
  dcaA(Ab)

SEQ ID NO: 186 - DNA, 1158 bp, Unknown
  Tfu1647
atgagtgacttcgacctctaccggcccaccgaggagcacgaagccctccgcgaagccatccgctccgtcgctgaagacaagatcgccccgcacgcggccgacgtcgacgagcagtcccgcttcccgcaggaggcctacgaggcgctgcgcgccagcgacttccacgctccccacgtcgcggaggagtacggcggtgttggcgcagacgcgctggcgacctgcatcgtcattgaggagatcgcccgggtgtgcgcctcctcttccctcatccccgcggtcaacaagctcggctcgatgccgctgatcctctccggatctgacgaggtgaagcagcgctacctgcccgaactggcatctggcgaggcgatgttctcctacgggctctccgagcgcgaggcgggatccgacaccgcgagcatgcgcacccgtgccgtccgcgacggcgacgactggatcctcaacggccagaagtcgtggatcacgaacgccggaatctccaagtactacacggtgatggcggtcaccgacccggacgggccgcgcggacgcaacatcagcgctttcgtcgtccacatcgacgatcccgggttctcttttggagaaccggaacgcaagctcggcatcaaaggttcgcccacgcgcgaactgatcttcgacaatgtccgtatccccggcgaccgcctggtgggcaaggtcggggaaggactgcgtaccgcgctgcgcaccctcgaccacacccgcgtcaccattggcgcccaggctgtgggcatcgcccagggggcgctcgactacgccctgggctatgtcaaggagcgcaagcagttcggcaaggccatcgccgacttccaaggcatccagttcatgctcgccgacatggccatgaagctggaagcggcccgccagatggtttacgtcgctgccgccaagtccgagcgcgacgacgccgacctctccttctacggtgccgccgctaaatgcttcgcctcggatgtggcaatggagatcaccactgacgcggtgcaactactcggcggctacggctacacccgggactacccggtcgagcggatgatgcgcgacgccaagatcacccagatctacgagggcaccaaccagatccagcgggtggtcatggcccggcagctcttgaagaagtga

SEQ ID NO: 187 - DNA, 873 bp, Unknown
  tesB(Ab)
atgaatacactaacccaagaactggttgaacttttatctctagaaaagctggaagagaacctctatcgcgggatgagccgaaatctggtggggaagcgcgtattcggtggtcaggttcttggacaagcattaagagctgcgtcatatacgacagatcgtcctgcacattcattacatgcttactttctctatggtggcgatgttaacgcccctattatttatgaagtagatcctttacgtgatggtaaaagttttgtgagtcgtcaggttcgcgctattcagcatggacgtactattttttctgcgatggtttcttttgcatcaccagaagaagggcttaactatcaaaatgatatgcctgattatcctgcacctgagcagcttaaatctgaagcggagttaaaactggggctgattgattttgtacctgaaaatgtacgtgccagttttatgcgtgaacgccacatagagattcgtccagttgagccagttaatccctttcagcctcaacctcaagcaccgactaacgcccactatatccgtacccatgacaagatcggaaaagcgtttgaccagattgcgctacaccagtctattgttgctttttattcagactttactttaatgacaacagcacttaaaccgcatggtttaagctatctttcaccgagtttgcagtgtgccagtatagatcacaccatttattttcatcgtccgttacgtgcagatgaatggatgctctacgacatggatgccacggtcagtgctggctcaagaggtttgaactttgggcgaatgtggcaaaatggattattggtttgtagcaccgtacaagaaggtttaatgcgccttcgtgaaattgaaacacagtaa

SEQ ID NO: 188 - DNA, 35 bp, Artificial Sequence; identical to SEQ ID NO: 34
  primer/ paaJ(Ec) IF

SEQ ID NO: 189 - DNA, 35 bp, Artificial Sequence; identical to SEQ ID NO: 35
  primer/ paaJ(Ec) IF

SEQ ID NO: 190 - DNA, 25 bp, Artificial Sequence
  primer/ pRSFDuet-P1
aagcttgcggccgcataatgcttaa

SEQ ID NO: 191 - DNA, 20 bp, Artificial Sequence
  primer/ pRSFDuet-P1
catggtatatctccttatta

SEQ ID NO: 192 - DNA, 35 bp, Artificial Sequence; identical to SEQ ID NO: 39
  primer/ paaH(Ec) IF

SEQ ID NO: 193 - DNA, 35 bp, Artificial Sequence; identical to SEQ ID NO: 40
  primer/ paaH(Ec) IF

SEQ ID NO: 194 - DNA, 25 bp, Artificial Sequence
  primer/ pRSFDuet-P2
ggtaccctcgagtctggtaaagaaa

SEQ ID NO: 195 - DNA, 20 bp, Artificial Sequence
  primer/ pRSFDuet-P2
catatgtatatctccttctt

SEQ ID NO: 196 - DNA, 35 bp, Artificial Sequence; identical to SEQ ID NO: 44
  primer/ paaF(Ec) IF

SEQ ID NO: 197 - DNA, 35 bp, Artificial Sequence; identical to SEQ ID NO: 45
  primer/ paaF(Ec) IF

SEQ ID NO: 198 - DNA, 35 bp, Artificial Sequence; identical to SEQ ID NO: 47
  primer/ paaF(L3)opt

SEQ ID NO: 199 - DNA, 35 bp, Artificial Sequence; identical to SEQ ID NO: 48
  primer/ paaF(L3)opt

SEQ ID NO: 200 - DNA, 35 bp, Artificial Sequence
  primer/ crt1(Ck)opt
agaaggagatataccatggaattcaagaacatcat

SEQ ID NO: 201 - DNA, 35 bp, Artificial Sequence
  primer/ crt1(Ck)opt
tgcggccgcaagcttttatttgtttttaaaggctt

SEQ ID NO: 202 - DNA, 35 bp, Artificial Sequence
  primer/ ech(Pp)opt
agaaggagatataccatgagcaaatatgaaggtcg

SEQ ID NO: 203 - DNA, 35 bp, Artificial Sequence
  primer/ ech(Pp)opt
tgcggccgcaagcttttaacgtttatatgcctgca

SEQ ID NO: 204 - DNA, 25 bp, Artificial Sequence
  primer/ pETDuet-P1
aagcttgcggccgcataatgcttaa

SEQ ID NO: 205 - DNA, 25 bp, Artificial Sequence
  primer/ pETDuet-P1
catggtatatctccttcttaaagtt

SEQ ID NO: 206 - DNA, 35 bp, Artificial Sequence; identical to SEQ ID NO: 52
  primer/ dcaA(Ab)

SEQ ID NO: 207 - DNA, 35 bp, Artificial Sequence; identical to SEQ ID NO: 53
  primer/ dcaA(Ab)

SEQ ID NO: 208 - DNA, 35 bp, Artificial Sequence
  primer/ Tfu1647
gaaggagatatacatatgagtgacttcgacctcta

SEQ ID NO: 209 - DNA, 35 bp, Artificial Sequence
  primer/ Tfu1647
tggcagcagcctaggtcacttcttcaagagctgcc

SEQ ID NO: 210 - DNA, 35 bp, Artificial Sequence
  rimer/ mmgC(L3)opt
gaaggagatatacatatgatccgtgatcaagaaac

SEQ ID NO: 211 - DNA, 35 bp, Artificial Sequence
  rimer/ mmgC(L3)opt
tggcagcagcctaggttacacctggacatcacgaa

SEQ ID NO: 212 - DNA, 25 bp, Artificial Sequence
  primer/ pETDuet-P2
cctaggctgctgccaccgctgagca

SEQ ID NO: 213 - DNA, 25 bp, Artificial Sequence
  primer/ pETDuet-P2
catatgtatatctccttcttatact

SEQ ID NO: 214 - DNA, 35 bp, Artificial Sequence
  primer/ tesB(Ab)
ataaggagatataccatgaatacactaacccaaga

SEQ ID NO: 215 - DNA, 35 bp, Artificial Sequence
  primer/ tesB(Ab)
tgcggccgcaagcttttactgtgtttcaatttcac

SEQ ID NO: 216 - DNA, 25 bp, Artificial Sequence
  primer/ pCDFDuet
aagcttgcggccgcataatgcttaa

SEQ ID NO: 217 - DNA, 20 bp, Artificial Sequence
  primer/ pCDFDuet
catggtatatctccttatta

SEQ ID NO: 218 - DNA, 35 bp, Artificial Sequence; identical to SEQ ID NO: 103
  primer/ ldh

SEQ ID NO: 219 - DNA, 35 bp, Artificial Sequence; identical to SEQ ID NO: 104
  primer/ ldh

SEQ ID NO: 220 - DNA, 35 bp, Artificial Sequence; identical to SEQ ID NO: 99
  primer/ atoB

SEQ ID NO: 221 - DNA, 35 bp, Artificial Sequence; identical to SEQ ID NO: 100
  primer/ atoB

SEQ ID NO: 222 - DNA, 35 bp, Artificial Sequence; identical to SEQ ID NO: 101
  primer/ sucD

SEQ ID NO: 223 - DNA, 35 bp, Artificial Sequence; identical to SEQ ID NO: 102
  primer/ sucD

SEQ ID NO: 224 - DNA, 35 bp, Artificial Sequence
  primer/ pHAK1
gatctgcatgcgatatctctagaacgcgtaagctt

SEQ ID NO: 225 - DNA, 29 bp, Artificial Sequence
  primer/ pHAK1
tctcgagccgatttattcaacaaagccgc

SEQ ID NO: 226 - DNA, 20 bp, Artificial Sequence
  primer/ del-ldh
tggtttaatcttgccgctcc

SEQ ID NO: 227 - DNA, 22 bp, Artificial Sequence
  primer/ del-ldh
gtgctataaacggcgagtttca

SEQ ID NO: 228 - DNA, 20 bp, Artificial Sequence
  primer/ del-atoB
cgatggtgattgaacggttg

SEQ ID NO: 229 - DNA, 20 bp, Artificial Sequence
  primer/ del-atoB
gcactgacgatgacacaatt

SEQ ID NO: 230 - DNA, 20 bp, Artificial Sequence
  primer/ del-sucD
gaaattcgctgctctggaag

SEQ ID NO: 231 - DNA, 23 bp, Artificial Sequence
  primer/ del-sucD
cctggcagataaccttggtgttt

SEQ ID NO: 232 - DNA, 35 bp, Artificial Sequence
  primer/ paaJ(L3)opt
ataaggagatataccatgctggatgcatatctgta

SEQ ID NO: 233 - DNA, 35 bp, Artificial Sequence
  primer/ paaJ(L3)opt
tgcggccgcaagcttttacatacgttcaataacaa

SEQ ID NO: 234 - DNA, 35 bp, Artificial Sequence
  primer/ paaH(L3)opt
gaaggagatatacatatgaacaccgatattcagac

SEQ ID NO: 235 - DNA, 35 bp, Artificial Sequence
  primer/ paaH(L3)opt
agactcgagggtaccttaattatccggtgtcagca

SEQ ID NO: 236 - protein, 453 aa, Clostridium kluyveri; identical to SEQ ID NO: 17

SEQ ID NO: 237 - protein, 1174 aa, Unknown; identical to SEQ ID NO: 18
  CAR

SEQ ID NO: 238 - protein, 1174 aa, Unknown; identical to SEQ ID NO: 19
  CAR

SEQ ID NO: 239 - protein, 1178 aa, Mycobacterium abscessus; identical to SEQ ID NO: 20

SEQ ID NO: 240 - protein, 1193 aa, Unknown; identical to SEQ ID NO: 21
  CAR

SEQ ID NO: 241 - protein, 1178 aa, Artificial Sequence; identical to SEQ ID NO: 22
  MaCar(m)

SEQ ID NO: 242 - protein, 224 aa, Unknown; identical to SEQ ID NO: 23
  PT

SEQ ID NO: 243 - protein, 222 aa, Nocardia iowensis; identical to SEQ ID NO: 24

SEQ ID NO: 244 - protein, 272 aa, Unknown; identical to SEQ ID NO: 25
  PT

SEQ ID NO: 245 - protein, 209 aa, Unknown; identical to SEQ ID NO: 26
  PT

SEQ ID NO: 246 - protein, 468 aa, Unknown; identical to SEQ ID NO: 27
  AT

SEQ ID NO: 247 - protein, 456 aa, Unknown; identical to SEQ ID NO: 28
  AT

SEQ ID NO: 248 - protein, 426 aa, Unknown; identical to SEQ ID NO: 29
  AT

SEQ ID NO: 249 - protein, 421 aa, Unknown; identical to SEQ ID NO: 30
  AT

SEQ ID NO: 250 - protein, 464 aa, Unknown; identical to SEQ ID NO: 31
  AT

SEQ ID NO: 251 - protein, 339 aa, Escherichia coli; identical to SEQ ID NO: 32